European Patent Application EP 4 382 605 A1, published June 12, 2024. Title: Nucleic acid construct utilizing SNARE. Applicant: 花王株式会社. The sequence listing filed with the application follows.

SEQUENCE LISTING (94 sequences)

SEQ ID NO: 1 - DNA, 663 bp, Homo sapiens
  source 1..663: mol_type = genomic DNA
atggcgattctttttgctgttgttgccagggggaccactatccttgccaaacatgcttggtgtggaggaaacttcctggaggtgacagagcagattctggctaagataccttctgaaaataacaaactaacgtactcacatggcaattatttgtttcattacatctgccaagacaggattgtatatctttgtatcactgatgatgattttgaacgttcccgagcctttaattttctgaatgagataaagaagaggttccagactacttacggttcaagagcacagacagcacttccatatgccatgaatagcgagttctcaagtgtcttagctgcacagctgaagcatcactctgagaataagggcctagacaaagtgatggagactcaagcccaagtggatgaactgaaaggaatcatggtcagaaacatagatctggtagctcagcgaggagaaagattggaattattgattgacaaaacagaaaatcttgtggattcttctgtcaccttcaaaactaccagcagaaatcttgctcgagccatgtgtatgaagaacctcaagctcactattatcatcatcatcgtatcaattgtgttcatctatatcattgtttcacctctctgtggtggatttacatggccaagctgtgtgaagaaatag

SEQ ID NO: 2 - DNA, 774 bp, Homo sapiens
  source 1..774: mol_type = genomic DNA
atggatcccctgttccagcaaacgcacaagcaggtccacgagatccagtcttgcatgggacgcctggagacggcagacaagcagtctgtgcacatagtagaaaacgaaatccaagcaagcatagaccagatattcagccgtctagaacgtctggagattttgtccagcaaggagccccctaacaaaaggcaaaatgccagacttcgggttgaccagttaaagtatgatgtccagcacctgcagactgcgctcagaaacttccagcatcggcgccatgcaagggagcagcaggagagacagcgagaagagcttctgtctcgaaccttcaccactaacgactctgacaccaccataccaatggacgaatcactgcagtttaactcctccctccagaaagttcacaacggcatggatgacctcattttagatgggcacaatattttagatggactgaggacccagagactgaccttgaaggggactcagaagaagatccttgacattgccaacatgctgggcttgtccaacacagtgatgcggctcatcgagaagcgggctttccaggacaagtactttatgatagagacaaggtctcaccatgttgcccagaatggacccgaactcctgagctcaagagatcctcctgcatcagcctcccgaagtgctgggattataggtatgagccaccaccctgacctccaaataccttttgaactcaggcttggatttgaactctggttctatcaactattagctgtgatttcagatcagtga

SEQ ID NO: 3 - DNA, 750 bp, Homo sapiens
  source 1..750: mol_type = genomic DNA
atgtctctcgaagaccccttttttgtagtccgaggcgaggtgcagaaggcggtgaacacggcccgcgggctgtaccagcgctggtgcgagctcctgcaggaaagcgcggcggtcggacgcgaggagctggactggacgaccaatgagctgcggaatggcctgcgcagcatcgagtgggacctcgaggacctggaagagaccatcggtatagtggaagccaacccaggcaagttcaagctcccagccggggacctgcaggagagaaaggtgttcgtggagcggatgcgagaggcagtccaggaaatgaaggaccatatggtcagcccaacagccgtagcatttttggagaggaataacagagagatactcgcaggcaagccagctgcccagaagtcacccagcgacctgctggatgccagcgcagtctcggccacatctcgctacatcgaggagcagcaggccacacagcagctgatcatggatgaacaggatcaacagctggagatggtgtctgggagcatccaggttctgaagcacatgtccggccgcgttggagaagagctggacgagcagggcatcatgctggatgccttcgcccaagagatggaccacacccagtcccgcatggacggggtcctcaggaagttggccaaagtatcccacatgacgagtgaccgccgacagtggtgtgccatcgccgtgctagtgggggtgcttctcctcgttctcatcttactattctctctctga

SEQ ID NO: 4 - DNA, 1008 bp, Homo sapiens
  source 1..1008: mol_type = genomic DNA
atggcggtggacatcacgctgctattccgggccagcgtcaagaccgtgaagacgcggaacaaggcgctgggagtggcggtgggcggcggggtcgatggcagccgggacgagctgttccgccggagcccccggcccaagggcgacttctccagccgggcccgcgaagtgatttctcacattggcaaactgagagattttcttctggaacacaggaaagattatattaatgcttatagccataccatgtctgaatatgggaggatgacagacacagaacgagaccagatagaccaggatgcccagatattcatgaggacctgttcagaagcaattcagcaactacgaacagaagctcacaaggagatacattcccagcaagtgaaggagcacaggaccgctgttttggatttcattgaagattacttgaaaagagtatgtaaactttactcagaacagagagccatccgagttaaaagagtggtggataagaaaagattatctaagctggaaccagaaccaaatacaaagacaagagaatccacatcttctgagaaagtttcacagagtccttcaaaagactctgaagaaaaccctgccactgaagaacgtccagaaaaaattttggctgaaacacaacctgaattgggaacgtggggagatggcaaaggcgaagatgagttatccccagaagaaatacaaatgtttgaacaggaaaatcagcgactaattggtgaaatgaacagcttgtttgatgaagtgaggcaaatcgaagggagagtggttgagatttccagactccaagagatattcacggaaaaggttttgcaacaggaagctgagattgacagcattcaccagttagttgtgggggcaactgaaaatatcaaggaaggcaacgaagacataagagaggccattaaaaacaacgctggcttccgcgtgtggatcctcttcttcctcgtgatgtgctccttctccttgctcttcctcgactggtacgacagctag

SEQ ID NO: 5 - DNA, 816 bp, Homo sapiens
  source 1..816: mol_type = genomic DNA
atggcggctccccaagacgtccacgtccggatctgtaaccaagagattgtcaaatttgacctggaggtgaaggcgcttattcaggatatccgtgattgttcaggacccttaagtgctcttactgaactgaatactaaagtaaaagagaaatttcaacagttgcgtcacagaatacagccagttctctatcaaagggcatttatttggactgcttccacatttttttttaagctaacttattccctgacagacttttcttcaactcagcatgacttcaactctccaactacacctgttaccttcagtgacctggagcagttggctaaagagcaagacaaagaatcagagaaacaacttctactccaggaagtggagaatcacaaaaagcagatgctcagcaatcaggcctcatggaggaaagctaatctcacctgcaaaattgcaatcgacaatctagagaaagcagaacttcttcagggaggagatctcttaaggcaaaggaaaaccaccaaagagagcctggcccagacatccagtaccatcactgagagcctcatggggatcagcaggatgatggcccagcaggtccagcagagcgaggaggccatgcagtctctagtcacttcttcacgaacgatcctggatgcaaatgaagaatttaagtccatgtcgggcaccatccagctgggccggaagcttatcacaaaatacaatcgccgggagctgacggacaagcttctcatcttccttgcgctagccctgtttcttgctacggtcctctatattgtgaaaaagcggctctttccatttttgtga

SEQ ID NO: 6 - DNA, 786 bp, Homo sapiens
  source 1..786: mol_type = genomic DNA
atgtcttacactccaggagttggtggtgaccccgcccagttggcccagaggatctcttctaacatccagaagatcacacagtgttctgtggaaatacaaagaactctgaatcaacttggaacacctcaagattcacctgaattgaggcaacagttgcaacagaagcagcagtatactaaccagcttgccaaagaaacagataagtacattaaagagtttggatctctgcccaccacccccagtgaacagcgtcaaaggaaaatacagaaggatcgcttagtggcagagttcacaacatcactgacaaacttccagaaggtccagaggcaggctgctgagcgagagaaagagtttgttgctcgagtaagagccagttccagagtgtctggcagttttcctgaggacagctcaaaagaaaggaatcttgtatcctgggaaagccaaactcaacctcaagtgcaggtgcaggatgaagaaattacagaggatgacctccgtcttattcatgagagagaatcttctatcaggcaacttgaagctgatattatggatattaatgaaatatttaaagatttgggaatgatgattcatgaacaaggagatgtaatagatagcatagaagccaatgtggaaaatgcagaggtgcacgttcagcaagcaaatcagcagctgtcaagggcagcagattatcagcgcaaatccagaaaaaccctgtgcatcatcattcttatccttgtcattggagttgcgattatcagtctcatcatatggggattgaaccactga

SEQ ID NO: 7 - DNA, 675 bp, Homo sapiens
  source 1..675: mol_type = genomic DNA
atgtcgtccgacttcgaaggttacgagcaggacttcgcggtgctcactgcagagatcaccagcaagattgcgagggtcccacgactcccgcctgatgaaaagaaacagatggttgcaaatgtggagaaacagcttgaagaagcgaaagaactgcttgaacagatggatttggaagtccgagagataccaccccaaagtcgagggatgtacagcaacagaatgagaagctacaaacaagaaatgggaaaactcgaaacagattttaaaaggtcacggatcgcctacagtgacgaagtacggaatgagctcctgggggatgatgggaattcctcagagaaccagttgataaaattacgtgaagagagggcacatctgctcgataacacagagaggctggaaaggtcatctcggagactagaggctggataccaaatagcagtggaaaccgagcaaattggtcaggagatgttggaaaaccttagtcatgacagagaaaagatacagcgagcacgtgaaagacttcgggaaacagatgctaatttgggaaaaagctccaggattctgacagggatgttgcgaagaatcatccagaaccgcatcctgctcgtcatcctagggatcatcgtggtcatcaccatcctgatggcgatcactttttctgtcagaagacactga

SEQ ID NO: 8 - DNA, 978 bp, Homo sapiens
  source 1..978: mol_type = genomic DNA
atggccaccaggcgtttaaccgacgctttcttgttgttgcggaataattccatccaaaaccggcagctgttagccgagcaagtgagtagtcacatcacctccagccctctgcattcacgtagcattgctgcggagctggacgagcttgctgatgaccgtatggcactggtgtcaggcatcagcttagatccagaagcagcgattggtgtgacaaaacggccacctcctaagtgggtggatggagtggatgaaattcagtatgatgttggccggattaagcagaagatgaaagaattggccagccttcatgacaagcatttaaacagacccaccctggatgacagcagcgaagaggaacatgccattgagataactacccaagagatcactcagctcttccacaggtgccagcgtgccgtgcaggccctgccgagccgggcccgggcctgctccgagcaggaggggcggctgcttgggaacgtggtggcctcgctggcgcaggccctgcaggaactctccaccagcttccggcacgcacagtcaggctacctcaaacgcatgaagaatcgagaggaaagatcccagcattttttcgacacatcagtaccactaatggatgatggagacgataacactctttaccatcggggttttacagaggaccagttagttctggtggagcagaacacactgatggtggaagagcgggaacgagagattcgccagattgtacagtccatttctgacctgaatgaaatattcagggacttaggggcgatgattgtagaacagggtacagtccttgacagaattgactataacgttgaacagtcctgtatcaaaactgaagatggtttgaaacagcttcacaaggcagaacagtatcaaaagaagaatcggaagatgcttgtgattttaatattatttgtcatcatcattgtgctcattgttgtcctcgttggcgtgaagtctcgataa

SEQ ID NO: 9 - DNA, 1068 bp, Homo sapiens
  source 1..1068: mol_type = genomic DNA
atgatcccgcggaaacgctacgggtctaagaacacggatcagggtgtctacctgggtctctcaaagacacaggtcctgtcccctgcaactgctggcagtagcagcagcgacatcgcccctctgccccccccagtgaccctcgtccctccccctcccgacaccatgtcctgccgggatcggacccaggagtttctgtctgcctgcaagtcgctgcagacccgtcagaatggaatccagacaaataagccagctttgcgtgctgtccgacaacgcagtgaattcaccctcatggccaagcgcattgggaaagaccttagcaacacatttgccaagctggagaagctgacaatcttggcaaagcgcaagtccctctttgatgataaagcagtggaaattgaagagctaacatatatcatcaaacaggacatcaatagcctcaacaaacaaattgctcagctccaggatttcgtgagagccaagggcagccagagtggccggcacctgcagacccactccaacaccattgtggtctccttgcagtcgaaactggcttctatgtccaatgacttcaaatcggttttagaagtgaggacagagaacctgaagcagcagaggagccggagagagcagttctcccgggcacctgtgtcagccctgccccttgcccctaaccacctgggcggtggtgctgtggttctgggggcagagtcccatgcctccaaggatgtcgccatcgacatgatggactctcggaccagccagcagctgcagctcattgacgagcaggattcctacatccagagtcgggcagacaccatgcagaacattgagtcgacaattgttgagttgggctccatctttcagcagttggcacacatggttaaggaacaggaggaaaccattcagaggatcgacgagaacgtgctaggagcccagctggacgttgaggccgcccattcagagatcctcaagtacttccagtctgtcacctccaaccggtggctcatggtcaaaatcttcctcatcctcattgtcttcttcatcatctttgtggtcttccttgcttga

SEQ ID NO: 10 - protein, 220 aa, Homo sapiens
MAILFAVVARGTTILAKHAWCGGNFLEVTEQILAKIPSENNKLTYSHGNYLFHYICQDRIVYLCITDDDFERSRAFNFLNEIKKRFQTTYGSRAQTALPYAMNSEFSSVLAAQLKHHSENKGLDKVMETQAQVDELKGIMVRNIDLVAQRGERLELLIDKTENLVDSSVTFKTTSRNLARAMCMKNLKLTIIIIIVSIVFIYIIVSPLCGGFTWPSCVKK

SEQ ID NO: 11 - protein, 257 aa, Homo sapiens
MDPLFQQTHKQVHEIQSCMGRLETADKQSVHIVENEIQASIDQIFSRLERLEILSSKEPPNKRQNARLRVDQLKYDVQHLQTALRNFQHRRHAREQQERQREELLSRTFTTNDSDTTIPMDESLQFNSSLQKVHNGMDDLILDGHNILDGLRTQRLTLKGTQKKILDIANMLGLSNTVMRLIEKRAFQDKYFMIETRSHHVAQNGPELLSSRDPPASASRSAGIIGMSHHPDLQIPFELRLGFELWFYQLLAVISDQ

SEQ ID NO: 12 - protein, 249 aa, Homo sapiens
MSLEDPFFVVRGEVQKAVNTARGLYQRWCELLQESAAVGREELDWTTNELRNGLRSIEWDLEDLEETIGIVEANPGKFKLPAGDLQERKVFVERMREAVQEMKDHMVSPTAVAFLERNNREILAGKPAAQKSPSDLLDASAVSATSRYIEEQQATQQLIMDEQDQQLEMVSGSIQVLKHMSGRVGEELDEQGIMLDAFAQEMDHTQSRMDGVLRKLAKVSHMTSDRRQWCAIAVLVGVLLLVLILLFSL

SEQ ID NO: 13 - protein, 335 aa, Homo sapiens
MAVDITLLFRASVKTVKTRNKALGVAVGGGVDGSRDELFRRSPRPKGDFSSRAREVISHIGKLRDFLLEHRKDYINAYSHTMSEYGRMTDTERDQIDQDAQIFMRTCSEAIQQLRTEAHKEIHSQQVKEHRTAVLDFIEDYLKRVCKLYSEQRAIRVKRVVDKKRLSKLEPEPNTKTRESTSSEKVSQSPSKDSEENPATEERPEKILAETQPELGTWGDGKGEDELSPEEIQMFEQENQRLIGEMNSLFDEVRQIEGRVVEISRLQEIFTEKVLQQEAEIDSIHQLVVGATENIKEGNEDIREAIKNNAGFRVWILFFLVMCSFSLLFLDWYDS

SEQ ID NO: 14 - protein, 271 aa, Homo sapiens
MAAPQDVHVRICNQEIVKFDLEVKALIQDIRDCSGPLSALTELNTKVKEKFQQLRHRIQPVLYQRAFIWTASTFFFKLTYSLTDFSSTQHDFNSPTTPVTFSDLEQLAKEQDKESEKQLLLQEVENHKKQMLSNQASWRKANLTCKIAIDNLEKAELLQGGDLLRQRKTTKESLAQTSSTITESLMGISRMMAQQVQQSEEAMQSLVTSSRTILDANEEFKSMSGTIQLGRKLITKYNRRELTDKLLIFLALALFLATVLYIVKKRLFPFL

SEQ ID NO: 15 - protein, 261 aa, Homo sapiens
MSYTPGVGGDPAQLAQRISSNIQKITQCSVEIQRTLNQLGTPQDSPELRQQLQQKQQYTNQLAKETDKYIKEFGSLPTTPSEQRQRKIQKDRLVAEFTTSLTNFQKVQRQAAEREKEFVARVRASSRVSGSFPEDSSKERNLVSWESQTQPQVQVQDEEITEDDLRLIHERESSIRQLEADIMDINEIFKDLGMMIHEQGDVIDSIEANVENAEVHVQQANQQLSRAADYQRKSRKTLCIIILILVIGVAIISLIIWGLNH

SEQ ID NO: 16 - protein, 224 aa, Homo sapiens
MSSDFEGYEQDFAVLTAEITSKIARVPRLPPDEKKQMVANVEKQLEEAKELLEQMDLEVREIPPQSRGMYSNRMRSYKQEMGKLETDFKRSRIAYSDEVRNELLGDDGNSSENQLIKLREERAHLLDNTERLERSSRRLEAGYQIAVETEQIGQEMLENLSHDREKIQRARERLRETDANLGKSSRILTGMLRRIIQNRILLVILGIIVVITILMAITFSVRRH

SEQ ID NO: 17 - protein, 325 aa, Homo sapiens
MATRRLTDAFLLLRNNSIQNRQLLAEQVSSHITSSPLHSRSIAAELDELADDRMALVSGISLDPEAAIGVTKRPPPKWVDGVDEIQYDVGRIKQKMKELASLHDKHLNRPTLDDSSEEEHAIEITTQEITQLFHRCQRAVQALPSRARACSEQEGRLLGNVVASLAQALQELSTSFRHAQSGYLKRMKNREERSQHFFDTSVPLMDDGDDNTLYHRGFTEDQLVLVEQNTLMVEEREREIRQIVQSISDLNEIFRDLGAMIVEQGTVLDRIDYNVEQSCIKTEDGLKQLHKAEQYQKKNRKMLVILILFVIIIVLIVVLVGVKSR

SEQ ID NO: 18 - protein, 355 aa, Homo sapiens
MIPRKRYGSKNTDQGVYLGLSKTQVLSPATAGSSSSDIAPLPPPVTLVPPPPDTMSCRDRTQEFLSACKSLQTRQNGIQTNKPALRAVRQRSEFTLMAKRIGKDLSNTFAKLEKLTILAKRKSLFDDKAVEIEELTYIIKQDINSLNKQIAQLQDFVRAKGSQSGRHLQTHSNTIVVSLQSKLASMSNDFKSVLEVRTENLKQQRSRREQFSRAPVSALPLAPNHLGGGAVVLGAESHASKDVAIDMMDSRTSQQLQLIDEQDSYIQSRADTMQNIESTIVELGSIFQQLAHMVKEQEETIQRIDENVLGAQLDVEAAHSEILKYFQSVTSNRWLMVKIFLILIVFFIIFVVFLA

SEQ ID NO: 19 - DNA, 45 bp, synthetic construct
  source 1..45: mol_type = other DNA; note = linker
ggcggcggaggatctggcggaggtggaagcggaggcggaggaagt

SEQ ID NO: 20 - protein, 15 aa, synthetic construct
  source 1..15: note = linker
GGGGSGGGGSGGGGS

SEQ ID NO: 21 - DNA, 15 bp, synthetic construct
  source 1..15: mol_type = other DNA; note = proprotein convertase (e.g., furin) recognition sequence
agaagggccagaaga

SEQ ID NO: 22 - protein, 5 aa, synthetic construct
  source 1..5: note = proprotein convertase (e.g., furin) recognition sequence
RRARR

SEQ ID NO: 23 - DNA, 1161 bp, Gallus gallus
  source 1..1161: mol_type = genomic DNA
atgggctccatcggcgcagcaagcatggaattttgttttgatgtattcaaggagctcaaagtccaccatgccaatgagaacatcttctactgccccattgccatcatgtcagctctagccatggtatacctgggtgcaaaagacagcaccaggacacagataaataaggttgttcgctttgataaacttccaggattcggagacagtattgaagctcagtgtggcacatctgtaaacgttcactcttcacttagagacatcctcaaccaaatcaccaaaccaaatgatgtttattcgttcagccttgccagtagactttatgctgaagagagatacccaatcctgccagaatacttgcagtgtgtgaaggaactgtatagaggaggcttggaacctatcaactttcaaacagctgcagatcaagccagagagctcatcaattcctgggtagaaagtcagacaaatggaattatcagaaatgtccttcagccaagctccgtggattctcaaactgcaatggttctggttaatgccattgtcttcaaaggactgtgggagaaaacatttaaggatgaagacacacaagcaatgcctttcagagtgactgagcaagaaagcaaacctgtgcagatgatgtaccagattggtttatttagagtggcatcaatggcttctgagaaaatgaagatcctggagcttccatttgccagtgggacaatgagcatgttggtgctgttgcctgatgaagtctcaggccttgagcagcttgagagtataatcaactttgaaaaactgactgaatggaccagttctaatgttatggaagagaggaagatcaaagtgtacttacctcgcatgaagatggaggaaaaatacaacctcacatctgtcttaatggctatgggcattactgacgtgtttagctcttcagccaatctgtctggcatctcctcagcagagagcctgaagatatctcaagctgtccatgcagcacatgcagaaatcaatgaagcaggcagagaggtggtagggtcagcagaggctggagtggatgctgcaagcgtctctgaagaatttagggctgaccatccattcctcttctgtatcaagcacatcgcaaccaacgccgttctcttctttggcagatgtgtttccccttaa

SEQ ID NO: 24 - protein, 386 aa, Gallus gallus
MGSIGAASMEFCFDVFKELKVHHANENIFYCPIAIMSALAMVYLGAKDSTRTQINKVVRFDKLPGFGDSIEAQCGTSVNVHSSLRDILNQITKPNDVYSFSLASRLYAEERYPILPEYLQCVKELYRGGLEPINFQTAADQARELINSWVESQTNGIIRNVLQPSSVDSQTAMVLVNAIVFKGLWEKTFKDEDTQAMPFRVTEQESKPVQMMYQIGLFRVASMASEKMKILELPFASGTMSMLVLLPDEVSGLEQLESIINFEKLTEWTSSNVMEERKIKVYLPRMKMEEKYNLTSVLMAMGITDVFSSSANLSGISSAESLKISQAVHAAHAEINEAGREVVGSAEAGVDAASVSEEFRADHPFLFCIKHIATNAVLFFGRCVSP

SEQ ID NO: 25 - protein, 621 aa, synthetic construct
  source 1..621: note = VAMP7-OVA
MAILFAVVARGTTILAKHAWCGGNFLEVTEQILAKIPSENNKLTYSHGNYLFHYICQDRIVYLCITDDDFERSRAFNFLNEIKKRFQTTYGSRAQTALPYAMNSEFSSVLAAQLKHHSENKGLDKVMETQAQVDELKGIMVRNIDLVAQRGERLELLIDKTENLVDSSVTFKTTSRNLARAMCMKNLKLTIIIIIVSIVFIYIIVSPLCGGFTWPSCVKKSGGGGSGGGGSGGGGSGSIGAASMEFCFDVFKELKVHHANENIFYCPIAIMSALAMVYLGAKDSTRTQINKVVRFDKLPGFGDSIEAQCGTSVNVHSSLRDILNQITKPNDVYSFSLASRLYAEERYPILPEYLQCVKELYRGGLEPINFQTAADQARELINSWVESQTNGIIRNVLQPSSVDSQTAMVLVNAIVFKGLWEKTFKDEDTQAMPFRVTEQESKPVQMMYQIGLFRVASMASEKMKILELPFASGTMSMLVLLPDEVSGLEQLESIINFEKLTEWTSSNVMEERKIKVYLPRMKMEEKYNLTSVLMAMGITDVFSSSANLSGISSAESLKISQAVHAAHAEINEAGREVVGSAEAGVDAASVSEEFRADHPFLFCIKHIATNAVLFFGRCVSP

SEQ ID NO: 26 - protein, 657 aa, synthetic construct
  source 1..657: note = GOSR2-OVA
MDPLFQQTHKQVHEIQSCMGRLETADKQSVHIVENEIQASIDQIFSRLERLEILSSKEPPNKRQNARLRVDQLKYDVQHLQTALRNFQHRRHAREQQERQREELLSRTFTTNDSDTTIPMDESLQFNSSLQKVHNGMDDLILDGHNILDGLRTQRLTLKGTQKKILDIANMLGLSNTVMRLIEKRAFQDKYFMIETRSHHVAQNGPELLSSRDPPASASRSAGIIGMSHHPDLQIPFELRLGFELWFYQLLAVISDQGGGGSGGGGSGGGGSGSIGAASMEFCFDVFKELKVHHANENIFYCPIAIMSALAMVYLGAKDSTRTQINKVVRFDKLPGFGDSIEAQCGTSVNVHSSLRDILNQITKPNDVYSFSLASRLYAEERYPILPEYLQCVKELYRGGLEPINFQTAADQARELINSWVESQTNGIIRNVLQPSSVDSQTAMVLVNAIVFKGLWEKTFKDEDTQAMPFRVTEQESKPVQMMYQIGLFRVASMASEKMKILELPFASGTMSMLVLLPDEVSGLEQLESIINFEKLTEWTSSNVMEERKIKVYLPRMKMEEKYNLTSVLMAMGITDVFSSSANLSGISSAESLKISQAVHAAHAEINEAGREVVGSAEAGVDAASVSEEFRADHPFLFCIKHIATNAVLFFGRCVSP

SEQ ID NO: 27 - protein, 649 aa, synthetic construct
  source 1..649: note = STX10-OVA
MSLEDPFFVVRGEVQKAVNTARGLYQRWCELLQESAAVGREELDWTTNELRNGLRSIEWDLEDLEETIGIVEANPGKFKLPAGDLQERKVFVERMREAVQEMKDHMVSPTAVAFLERNNREILAGKPAAQKSPSDLLDASAVSATSRYIEEQQATQQLIMDEQDQQLEMVSGSIQVLKHMSGRVGEELDEQGIMLDAFAQEMDHTQSRMDGVLRKLAKVSHMTSDRRQWCAIAVLVGVLLLVLILLFSLGGGGSGGGGSGGGGSGSIGAASMEFCFDVFKELKVHHANENIFYCPIAIMSALAMVYLGAKDSTRTQINKVVRFDKLPGFGDSIEAQCGTSVNVHSSLRDILNQITKPNDVYSFSLASRLYAEERYPILPEYLQCVKELYRGGLEPINFQTAADQARELINSWVESQTNGIIRNVLQPSSVDSQTAMVLVNAIVFKGLWEKTFKDEDTQAMPFRVTEQESKPVQMMYQIGLFRVASMASEKMKILELPFASGTMSMLVLLPDEVSGLEQLESIINFEKLTEWTSSNVMEERKIKVYLPRMKMEEKYNLTSVLMAMGITDVFSSSANLSGISSAESLKISQAVHAAHAEINEAGREVVGSAEAGVDAASVSEEFRADHPFLFCIKHIATNAVLFFGRCVSP

SEQ ID NO: 28 - protein, 735 aa, synthetic construct
  source 1..735: note = STX18-OVA
MAVDITLLFRASVKTVKTRNKALGVAVGGGVDGSRDELFRRSPRPKGDFSSRAREVISHIGKLRDFLLEHRKDYINAYSHTMSEYGRMTDTERDQIDQDAQIFMRTCSEAIQQLRTEAHKEIHSQQVKEHRTAVLDFIEDYLKRVCKLYSEQRAIRVKRVVDKKRLSKLEPEPNTKTRESTSSEKVSQSPSKDSEENPATEERPEKILAETQPELGTWGDGKGEDELSPEEIQMFEQENQRLIGEMNSLFDEVRQIEGRVVEISRLQEIFTEKVLQQEAEIDSIHQLVVGATENIKEGNEDIREAIKNNAGFRVWILFFLVMCSFSLLFLDWYDSGGGGSGGGGSGGGGSGSIGAASMEFCFDVFKELKVHHANENIFYCPIAIMSALAMVYLGAKDSTRTQINKVVRFDKLPGFGDSIEAQCGTSVNVHSSLRDILNQITKPNDVYSFSLASRLYAEERYPILPEYLQCVKELYRGGLEPINFQTAADQARELINSWVESQTNGIIRNVLQPSSVDSQTAMVLVNAIVFKGLWEKTFKDEDTQAMPFRVTEQESKPVQMMYQIGLFRVASMASEKMKILELPFASGTMSMLVLLPDEVSGLEQLESIINFEKLTEWTSSNVMEERKIKVYLPRMKMEEKYNLTSVLMAMGITDVFSSSANLSGISSAESLKISQAVHAAHAEINEAGREVVGSAEAGVDAASVSEEFRADHPFLFCIKHIATNAVLFFGRCVSP

SEQ ID NO: 29 - protein, 671 aa, synthetic construct
  source 1..671: note = BNIP1-OVA
MAAPQDVHVRICNQEIVKFDLEVKALIQDIRDCSGPLSALTELNTKVKEKFQQLRHRIQPVLYQRAFIWTASTFFFKLTYSLTDFSSTQHDFNSPTTPVTFSDLEQLAKEQDKESEKQLLLQEVENHKKQMLSNQASWRKANLTCKIAIDNLEKAELLQGGDLLRQRKTTKESLAQTSSTITESLMGISRMMAQQVQQSEEAMQSLVTSSRTILDANEEFKSMSGTIQLGRKLITKYNRRELTDKLLIFLALALFLATVLYIVKKRLFPFLGGGGSGGGGSGGGGSGSIGAASMEFCFDVFKELKVHHANENIFYCPIAIMSALAMVYLGAKDSTRTQINKVVRFDKLPGFGDSIEAQCGTSVNVHSSLRDILNQITKPNDVYSFSLASRLYAEERYPILPEYLQCVKELYRGGLEPINFQTAADQARELINSWVESQTNGIIRNVLQPSSVDSQTAMVLVNAIVFKGLWEKTFKDEDTQAMPFRVTEQESKPVQMMYQIGLFRVASMASEKMKILELPFASGTMSMLVLLPDEVSGLEQLESIINFEKLTEWTSSNVMEERKIKVYLPRMKMEEKYNLTSVLMAMGITDVFSSSANLSGISSAESLKISQAVHAAHAEINEAGREVVGSAEAGVDAASVSEEFRADHPFLFCIKHIATNAVLFFGRCVSP

SEQ ID NO: 30 - protein, 661 aa, synthetic construct
  source 1..661: note = STX7-OVA
MSYTPGVGGDPAQLAQRISSNIQKITQCSVEIQRTLNQLGTPQDSPELRQQLQQKQQYTNQLAKETDKYIKEFGSLPTTPSEQRQRKIQKDRLVAEFTTSLTNFQKVQRQAAEREKEFVARVRASSRVSGSFPEDSSKERNLVSWESQTQPQVQVQDEEITEDDLRLIHERESSIRQLEADIMDINEIFKDLGMMIHEQGDVIDSIEANVENAEVHVQQANQQLSRAADYQRKSRKTLCIIILILVIGVAIISLIIWGLNHGGGGSGGGGSGGGGSGSIGAASMEFCFDVFKELKVHHANENIFYCPIAIMSALAMVYLGAKDSTRTQINKVVRFDKLPGFGDSIEAQCGTSVNVHSSLRDILNQITKPNDVYSFSLASRLYAEERYPILPEYLQCVKELYRGGLEPINFQTAADQARELINSWVESQTNGIIRNVLQPSSVDSQTAMVLVNAIVFKGLWEKTFKDEDTQAMPFRVTEQESKPVQMMYQIGLFRVASMASEKMKILELPFASGTMSMLVLLPDEVSGLEQLESIINFEKLTEWTSSNVMEERKIKVYLPRMKMEEKYNLTSVLMAMGITDVFSSSANLSGISSAESLKISQAVHAAHAEINEAGREVVGSAEAGVDAASVSEEFRADHPFLFCIKHIATNAVLFFGRCVSP

SEQ ID NO: 31 - protein, 624 aa, synthetic construct
  source 1..624: note = VTI1A-OVA
MSSDFEGYEQDFAVLTAEITSKIARVPRLPPDEKKQMVANVEKQLEEAKELLEQMDLEVREIPPQSRGMYSNRMRSYKQEMGKLETDFKRSRIAYSDEVRNELLGDDGNSSENQLIKLREERAHLLDNTERLERSSRRLEAGYQIAVETEQIGQEMLENLSHDREKIQRARERLRETDANLGKSSRILTGMLRRIIQNRILLVILGIIVVITILMAITFSVRRHGGGGSGGGGSGGGGSGSIGAASMEFCFDVFKELKVHHANENIFYCPIAIMSALAMVYLGAKDSTRTQINKVVRFDKLPGFGDSIEAQCGTSVNVHSSLRDILNQITKPNDVYSFSLASRLYAEERYPILPEYLQCVKELYRGGLEPINFQTAADQARELINSWVESQTNGIIRNVLQPSSVDSQTAMVLVNAIVFKGLWEKTFKDEDTQAMPFRVTEQESKPVQMMYQIGLFRVASMASEKMKILELPFASGTMSMLVLLPDEVSGLEQLESIINFEKLTEWTSSNVMEERKIKVYLPRMKMEEKYNLTSVLMAMGITDVFSSSANLSGISSAESLKISQAVHAAHAEINEAGREVVGSAEAGVDAASVSEEFRADHPFLFCIKHIATNAVLFFGRCVSP

SEQ ID NO: 32 - protein, 725 aa, synthetic construct
  source 1..725: note = STX16-OVA
MATRRLTDAFLLLRNNSIQNRQLLAEQVSSHITSSPLHSRSIAAELDELADDRMALVSGISLDPEAAIGVTKRPPPKWVDGVDEIQYDVGRIKQKMKELASLHDKHLNRPTLDDSSEEEHAIEITTQEITQLFHRCQRAVQALPSRARACSEQEGRLLGNVVASLAQALQELSTSFRHAQSGYLKRMKNREERSQHFFDTSVPLMDDGDDNTLYHRGFTEDQLVLVEQNTLMVEEREREIRQIVQSISDLNEIFRDLGAMIVEQGTVLDRIDYNVEQSCIKTEDGLKQLHKAEQYQKKNRKMLVILILFVIIIVLIVVLVGVKSRGGGGSGGGGSGGGGSGSIGAASMEFCFDVFKELKVHHANENIFYCPIAIMSALAMVYLGAKDSTRTQINKVVRFDKLPGFGDSIEAQCGTSVNVHSSLRDILNQITKPNDVYSFSLASRLYAEERYPILPEYLQCVKELYRGGLEPINFQTAADQARELINSWVESQTNGIIRNVLQPSSVDSQTAMVLVNAIVFKGLWEKTFKDEDTQAMPFRVTEQESKPVQMMYQIGLFRVASMASEKMKILELPFASGTMSMLVLLPDEVSGLEQLESIINFEKLTEWTSSNVMEERKIKVYLPRMKMEEKYNLTSVLMAMGITDVFSSSANLSGISSAESLKISQAVHAAHAEINEAGREVVGSAEAGVDAASVSEEFRADHPFLFCIKHIATNAVLFFGRCVSP

SEQ ID NO: 33 - protein, 755 aa, synthetic construct
  source 1..755: note = STX5-OVA
MIPRKRYGSKNTDQGVYLGLSKTQVLSPATAGSSSSDIAPLPPPVTLVPPPPDTMSCRDRTQEFLSACKSLQTRQNGIQTNKPALRAVRQRSEFTLMAKRIGKDLSNTFAKLEKLTILAKRKSLFDDKAVEIEELTYIIKQDINSLNKQIAQLQDFVRAKGSQSGRHLQTHSNTIVVSLQSKLASMSNDFKSVLEVRTENLKQQRSRREQFSRAPVSALPLAPNHLGGGAVVLGAESHASKDVAIDMMDSRTSQQLQLIDEQDSYIQSRADTMQNIESTIVELGSIFQQLAHMVKEQEETIQRIDENVLGAQLDVEAAHSEILKYFQSVTSNRWLMVKIFLILIVFFIIFVVFLAGGGGSGGGGSGGGGSGSIGAASMEFCFDVFKELKVHHANENIFYCPIAIMSALAMVYLGAKDSTRTQINKVVRFDKLPGFGDSIEAQCGTSVNVHSSLRDILNQITKPNDVYSFSLASRLYAEERYPILPEYLQCVKELYRGGLEPINFQTAADQARELINSWVESQTNGIIRNVLQPSSVDSQTAMVLVNAIVFKGLWEKTFKDEDTQAMPFRVTEQESKPVQMMYQIGLFRVASMASEKMKILELPFASGTMSMLVLLPDEVSGLEQLESIINFEKLTEWTSSNVMEERKIKVYLPRMKMEEKYNLTSVLMAMGITDVFSSSANLSGISSAESLKISQAVHAAHAEINEAGREVVGSAEAGVDAASVSEEFRADHPFLFCIKHIATNAVLFFGRCVSP

SEQ ID NO: 34 - protein, 655 aa, synthetic construct
  source 1..655: note = STX6-OVA
MSMEDPFFVVKGEVQKAVNTAQGLFQRWTELLQDPSTATREEIDWTTNELRNNLRSIEWDLEDLDETISIVEANPRKFNLDATELSIRKAFITSTRQVVRDMKDQMSTSSVQALAERKNRQALLGDSGSQNWSTGTTDKYGRLDRELQRANSHFIEEQQAQQQLIVEQQDEQLELVSGSIGVLKNMSQRIGGELEEQAVMLEDFSHELESTQSRLDNVMKKLAKVSHMTSDRRQWCAIAILFAVLLVVLILFLVLGGGGSGGGGSGGGGSGSIGAASMEFCFDVFKELKVHHANENIFYCPIAIMSALAMVYLGAKDSTRTQINKVVRFDKLPGFGDSIEAQCGTSVNVHSSLRDILNQITKPNDVYSFSLASRLYAEERYPILPEYLQCVKELYRGGLEPINFQTAADQARELINSWVESQTNGIIRNVLQPSSVDSQTAMVLVNAIVFKGLWEKTFKDEDTQAMPFRVTEQESKPVQMMYQIGLFRVASMASEKMKILELPFASGTMSMLVLLPDEVSGLEQLESIINFEKLTEWTSSNVMEERKIKVYLPRMKMEEKYNLTSVLMAMGITDVFSSSANLSGISSAESLKISQAVHAAHAEINEAGREVVGSAEAGVDAASVSEEFRADHPFLFCIKHIATNAVLFFGRCVSP

SEQ ID NO: 35 - protein, 636 aa, synthetic construct
  source 1..636: note = STX8-OVA
MAPDPWFSTYDSTCQIAQEIAEKIQQRNQYERKGEKAPKLTVTIRALLQNLKEKIALLKDLLLRAVSTHQITQLEGDRRQNLLDDLVTRERLLLASFKNEGAEPDLIRSSLMSEEAKRGAPNPWLFEEPEETRGLGFDEIRQQQQKIIQEQDAGLDALSSIISRQKQMGQEIGNELDEQNEIIDDLANLVENTDEKLRNETRRVNMVDRKSASCGMIMVILLLLVAIVVVAVWPTNGGGGSGGGGSGGGGSGSIGAASMEFCFDVFKELKVHHANENIFYCPIAIMSALAMVYLGAKDSTRTQINKVVRFDKLPGFGDSIEAQCGTSVNVHSSLRDILNQITKPNDVYSFSLASRLYAEERYPILPEYLQCVKELYRGGLEPINFQTAADQARELINSWVESQTNGIIRNVLQPSSVDSQTAMVLVNAIVFKGLWEKTFKDEDTQAMPFRVTEQESKPVQMMYQIGLFRVASMASEKMKILELPFASGTMSMLVLLPDEVSGLEQLESIINFEKLTEWTSSNVMEERKIKVYLPRMKMEEKYNLTSVLMAMGITDVFSSSANLSGISSAESLKISQAVHAAHAEINEAGREVVGSAEAGVDAASVSEEFRADHPFLFCIKHIATNAVLFFGRCVSP

SEQ ID NO: 36 - protein, 676 aa, synthetic construct
  source 1..676: note = STX12-OVA
MSYGPLDMYRNPGPSGPQLRDFSSIIQTCSGNIQRISQATAQIKNLMSQLGTKQDSSKLQENLQQLQHSTNQLAKETNELLKELGSLPLPLSTSEQRQQRLQKERLMNDFSAALNNFQAVQRRVSEKEKESIARARAGSRLSAEERQREEQLVSFDSHEEWNQMQSQEDEVAITEQDLELIKERETAIRQLEADILDVNQIFKDLAMMIHDQGDLIDSIEANVESSEVHVERATEQLQRAAYYQKKSRKKMCILVLVLSVIILILGLIIWLVYKTKGGGGSGGGGSGGGGSGSIGAASMEFCFDVFKELKVHHANENIFYCPIAIMSALAMVYLGAKDSTRTQINKVVRFDKLPGFGDSIEAQCGTSVNVHSSLRDILNQITKPNDVYSFSLASRLYAEERYPILPEYLQCVKELYRGGLEPINFQTAADQARELINSWVESQTNGIIRNVLQPSSVDSQTAMVLVNAIVFKGLWEKTFKDEDTQAMPFRVTEQESKPVQMMYQIGLFRVASMASEKMKILELPFASGTMSMLVLLPDEVSGLEQLESIINFEKLTEWTSSNVMEERKIKVYLPRMKMEEKYNLTSVLMAMGITDVFSSSANLSGISSAESLKISQAVHAAHAEINEAGREVVGSAEAGVDAASVSEEFRADHPFLFCIKHIATNAVLFFGRCVSP

SEQ ID NO: 37 - protein, 500 aa, synthetic construct
  source 1..500: note = VAMP3-OVA
MSTGPTAATGSNRRLQQTQNQVDEVVDIMRVNVDKVLERDQKLSELDDRADALQAGASQFETSAAKLKRKYWWKNCKMWAIGITVLVIFIIIIIVWVVSSGGGGSGGGGSGGGGSGSIGAASMEFCFDVFKELKVHHANENIFYCPIAIMSALAMVYLGAKDSTRTQINKVVRFDKLPGFGDSIEAQCGTSVNVHSSLRDILNQITKPNDVYSFSLASRLYAEERYPILPEYLQCVKELYRGGLEPINFQTAADQARELINSWVESQTNGIIRNVLQPSSVDSQTAMVLVNAIVFKGLWEKTFKDEDTQAMPFRVTEQESKPVQMMYQIGLFRVASMASEKMKILELPFASGTMSMLVLLPDEVSGLEQLESIINFEKLTEWTSSNVMEERKIKVYLPRMKMEEKYNLTSVLMAMGITDVFSSSANLSGISSAESLKISQAVHAAHAEINEAGREVVGSAEAGVDAASVSEEFRADHPFLFCIKHIATNAVLFFGRCVSP

SEQ ID NO: 38 - protein, 541 aa, synthetic construct
  source 1..541: note = VAMP4-OVA
MPPKFKRHLNDDDVTGSVKSERRNLLEDDSDEEEDFFLRGPSGPRFGPRNDKIKHVQNQVDEVIDVMQENITKVIERGERLDELQDKSESLSDNATAFSNRSKQLRRQMWWRGCKIKAIMALVAAILLLVIIILIVMKYRTGGGGSGGGGSGGGGSGSIGAASMEFCFDVFKELKVHHANENIFYCPIAIMSALAMVYLGAKDSTRTQINKVVRFDKLPGFGDSIEAQCGTSVNVHSSLRDILNQITKPNDVYSFSLASRLYAEERYPILPEYLQCVKELYRGGLEPINFQTAADQARELINSWVESQTNGIIRNVLQPSSVDSQTAMVLVNAIVFKGLWEKTFKDEDTQAMPFRVTEQESKPVQMMYQIGLFRVASMASEKMKILELPFASGTMSMLVLLPDEVSGLEQLESIINFEKLTEWTSSNVMEERKIKVYLPRMKMEEKYNLTSVLMAMGITDVFSSSANLSGISSAESLKISQAVHAAHAEINEAGREVVGSAEAGVDAASVSEEFRADHPFLFCIKHIATNAVLFFGRCVSP

SEQ ID NO: 39 - protein, 500 aa, synthetic construct
  source 1..500: note = VAMP8-OVA
MEEASEGGGNDRVRNLQSEVEGVKNIMTQNVERILARGENLEHLRNKTEDLEATSEHFKTTSQKVARKFWWKNVKMIVLICVIVFIIILFIVLFATGAFSGGGGSGGGGSGGGGSGSIGAASMEFCFDVFKELKVHHANENIFYCPIAIMSALAMVYLGAKDSTRTQINKVVRFDKLPGFGDSIEAQCGTSVNVHSSLRDILNQITKPNDVYSFSLASRLYAEERYPILPEYLQCVKELYRGGLEPINFQTAADQARELINSWVESQTNGIIRNVLQPSSVDSQTAMVLVNAIVFKGLWEKTFKDEDTQAMPFRVTEQESKPVQMMYQIGLFRVASMASEKMKILELPFASGTMSMLVLLPDEVSGLEQLESIINFEKLTEWTSSNVMEERKIKVYLPRMKMEEKYNLTSVLMAMGITDVFSSSANLSGISSAESLKISQAVHAAHAEINEAGREVVGSAEAGVDAASVSEEFRADHPFLFCIKHIATNAVLFFGRCVSP

SEQ ID NO: 40 - protein, 632 aa, synthetic construct
  source 1..632: note = VTI1B-OVA
MASSAASSEHFEKLHEIFRGLHEDLQGVPERLLGTAGTEEKKKLIRDFDEKQQEANETLAEMEEELRYAPLSFRNPMMSKLRNYRKDLAKLHREVRSTPLTATPGGRGDMKYGIYAVENEHMNRLQSQRAMLLQGTESLNRATQSIERSHRIATETDQIGSEIIEELGEQRDQLERTKSRLVNTSENLSKSRKILRSMSRKVTTNKLLLSIIILLELAILGGLVYYKFFRSHGGGGSGGGGSGGGGSGSIGAASMEFCFDVFKELKVHHANENIFYCPIAIMSALAMVYLGAKDSTRTQINKVVRFDKLPGFGDSIEAQCGTSVNVHSSLRDILNQITKPNDVYSFSLASRLYAEERYPILPEYLQCVKELYRGGLEPINFQTAADQARELINSWVESQTNGIIRNVLQPSSVDSQTAMVLVNAIVFKGLWEKTFKDEDTQAMPFRVTEQESKPVQMMYQIGLFRVASMASEKMKILELPFASGTMSMLVLLPDEVSGLEQLESIINFEKLTEWTSSNVMEERKIKVYLPRMKMEEKYNLTSVLMAMGITDVFSSSANLSGISSAESLKISQAVHAAHAEINEAGREVVGSAEAGVDAASVSEEFRADHPFLFCIKHIATNAVLFFGRCVSP

SEQ ID NO: 41 - protein, 650 aa, synthetic construct
  source 1..650: note = GOSR1-OVA
MAAGTSSYWEDLRKQARQLENELDLKLVSFSKLCTSYSHSSTRDGRRDRYSSDTTPLLNGSSQDRMFETMAIEIEQLLARLTGVNDKMAEYTNSAGVPSLNAALMHTLQRHRDILQDYTHEFHKTKANFMAIRERENLMGSVRKDIESYKSGSGVNNRRTELFLKEHDHLRNSDRLIEETISIAMATKENMTSQRGMLKSIHSKMNTLANRFPAVNSLIQRINLRKRRDSLILGGVIGICTILLLLYAFHGGGGSGGGGSGGGGSGSIGAASMEFCFDVFKELKVHHANENIFYCPIAIMSALAMVYLGAKDSTRTQINKVVRFDKLPGFGDSIEAQCGTSVNVHSSLRDILNQITKPNDVYSFSLASRLYAEERYPILPEYLQCVKELYRGGLEPINFQTAADQARELINSWVESQTNGIIRNVLQPSSVDSQTAMVLVNAIVFKGLWEKTFKDEDTQAMPFRVTEQESKPVQMMYQIGLFRVASMASEKMKILELPFASGTMSMLVLLPDEVSGLEQLESIINFEKLTEWTSSNVMEERKIKVYLPRMKMEEKYNLTSVLMAMGITDVFSSSANLSGISSAESLKISQAVHAAHAEINEAGREVVGSAEAGVDAASVSEEFRADHPFLFCIKHIATNAVLFFGRCVSP

SEQ ID NO: 42 - protein, 518 aa, synthetic construct
  source 1..518: note = BET1-OVA
MRRAGLGEGVPPGNYGNYGYANSGYSACEEENERLTESLRSKVTAIKSLSIEIGHEVKTQNKLLAEMDSQFDSTTGFLGKTMGKLKILSRGSQTKLLCYMMLFSLFVFFIIYWIIKLRGGGGSGGGGSGGGGSGSIGAASMEFCFDVFKELKVHHANENIFYCPIAIMSALAMVYLGAKDSTRTQINKVVRFDKLPGFGDSIEAQCGTSVNVHSSLRDILNQITKPNDVYSFSLASRLYAEERYPILPEYLQCVKELYRGGLEPINFQTAADQARELINSWVESQTNGIIRNVLQPSSVDSQTAMVLVNAIVFKGLWEKTFKDEDTQAMPFRVTEQESKPVQMMYQIGLFRVASMASEKMKILELPFASGTMSMLVLLPDEVSGLEQLESIINFEKLTEWTSSNVMEERKIKVYLPRMKMEEKYNLTSVLMAMGITDVFSSSANLSGISSAESLKISQAVHAAHAEINEAGREVVGSAEAGVDAASVSEEFRADHPFLFCIKHIATNAVLFFGRCVSP

SEQ ID NO: 43 - protein, 690 aa, synthetic construct
  source 1..690: note = BET1L-OVA
MAFCAILLVPSLCRMPSLPTSPWAFPVHWAGFMFKPLDWQGNDFFPPQDEVLAPCLGIKTPLKHEPCASLPFSVLFQSSASQSLLGTMGSLSPHLCGHTMCPVNPELPLSFQADHRSAQPDACSPLCHPSSLLPSFHTASLPFSIHAHHSPLPCDLDPPLYLAETVSLLEEWGPPSSCPMQCKLTSHPARLTHLPPCLWGFAVALKPSWAGLAPSLLPPPRMSLCRPLSFLRHQCPWLPWQAHQGLVPWSPSMVAAACIVSPSGHCRCQPFIPHVFLGHGGLTSVSGECGGGGGSGGGGSGGGGSGSIGAASMEFCFDVFKELKVHHANENIFYCPIAIMSALAMVYLGAKDSTRTQINKVVRFDKLPGFGDSIEAQCGTSVNVHSSLRDILNQITKPNDVYSFSLASRLYAEERYPILPEYLQCVKELYRGGLEPINFQTAADQARELINSWVESQTNGIIRNVLQPSSVDSQTAMVLVNAIVFKGLWEKTFKDEDTQAMPFRVTEQESKPVQMMYQIGLFRVASMASEKMKILELPFASGTMSMLVLLPDEVSGLEQLESIINFEKLTEWTSSNVMEERKIKVYLPRMKMEEKYNLTSVLMAMGITDVFSSSANLSGISSAESLKISQAVHAAHAEINEAGREVVGSAEAGVDAASVSEEFRADHPFLFCIKHIATNAVLFFGRCVSP

SEQ ID NO: 44 - protein, 615 aa, synthetic construct
  source 1..615: note = SEC22B-OVA
MVLLTMIARVADGLPLAASMQEDEQSGRDLQQYQSQAKQLFRKLNEQSPTRCTLEAGAMTFHYIIEQGVCYLVLCEAAFPKKLAFAYLEDLHSEFDEQHGKKVPTVSRPYSFIEFDTFIQKTKKLYIDSRARRNLGSINTELQDVQRIMVANIEEVLQRGEALSALDSKANNLSSLSKKYRQDAKYLNMRSTYAKLAAVAVFFIMLIVYVRFWWLGGGGSGGGGSGGGGSGSIGAASMEFCFDVFKELKVHHANENIFYCPIAIMSALAMVYLGAKDSTRTQINKVVRFDKLPGFGDSIEAQCGTSVNVHSSLRDILNQITKPNDVYSFSLASRLYAEERYPILPEYLQCVKELYRGGLEPINFQTAADQARELINSWVESQTNGIIRNVLQPSSVDSQTAMVLVNAIVFKGLWEKTFKDEDTQAMPFRVTEQESKPVQMMYQIGLFRVASMASEKMKILELPFASGTMSMLVLLPDEVSGLEQLESIINFEKLTEWTSSNVMEERKIKVYLPRMKMEEKYNLTSVLMAMGITDVFSSSANLSGISSAESLKISQAVHAAHAEINEAGREVVGSAEAGVDAASVSEEFRADHPFLFCIKHIATNAVLFFGRCVSP

SEQ ID NO: 45 - protein, 659 aa, synthetic construct
  source 1..659: note = USE1-OVA
MAASRLELNLVRLLSRCEAMAAEKRDPDEWRLEKYVGALEDMLQALKVHASKPASEVINEYSWKVDFLKGMLQAEKLTSSSEKALANQFLAPGRVPTTARERVPATKTVHLQSRARYTSEMRSELLGTDSAEPEMDVRKRTGVAGSQPVSEKQLAAELDLVLQRHQNLQEKLAEEMLGLARSLKTNTLAAQSVIKKDNQTLSHSLKMADQNLEKLKTESERLEQHTQKSVNWLLWAMLIIVCFIFISMILFIRIMPKLKGGGGSGGGGSGGGGSGSIGAASMEFCFDVFKELKVHHANENIFYCPIAIMSALAMVYLGAKDSTRTQINKVVRFDKLPGFGDSIEAQCGTSVNVHSSLRDILNQITKPNDVYSFSLASRLYAEERYPILPEYLQCVKELYRGGLEPINFQTAADQARELINSWVESQTNGIIRNVLQPSSVDSQTAMVLVNAIVFKGLWEKTFKDEDTQAMPFRVTEQESKPVQMMYQIGLFRVASMASEKMKILELPFASGTMSMLVLLPDEVSGLEQLESIINFEKLTEWTSSNVMEERKIKVYLPRMKMEEKYNLTSVLMAMGITDVFSSSANLSGISSAESLKISQAVHAAHAEINEAGREVVGSAEAGVDAASVSEEFRADHPFLFCIKHIATNAVLFFGRCVSP

SEQ ID NO: 46 - protein, 626 aa, synthetic construct
  source 1..626: note = VAMP7-pc-OVA
MAILFAVVARGTTILAKHAWCGGNFLEVTEQILAKIPSENNKLTYSHGNYLFHYICQDRIVYLCITDDDFERSRAFNFLNEIKKRFQTTYGSRAQTALPYAMNSEFSSVLAAQLKHHSENKGLDKVMETQAQVDELKGIMVRNIDLVAQRGERLELLIDKTENLVDSSVTFKTTSRNLARAMCMKNLKLTIIIIIVSIVFIYIIVSPLCGGFTWPSCVKKSGGGGSGGGGSGGGGSRRARRGSIGAASMEFCFDVFKELKVHHANENIFYCPIAIMSALAMVYLGAKDSTRTQINKVVRFDKLPGFGDSIEAQCGTSVNVHSSLRDILNQITKPNDVYSFSLASRLYAEERYPILPEYLQCVKELYRGGLEPINFQTAADQARELINSWVESQTNGIIRNVLQPSSVDSQTAMVLVNAIVFKGLWEKTFKDEDTQAMPFRVTEQESKPVQMMYQIGLFRVASMASEKMKILELPFASGTMSMLVLLPDEVSGLEQLESIINFEKLTEWTSSNVMEERKIKVYLPRMKMEEKYNLTSVLMAMGITDVFSSSANLSGISSAESLKISQAVHAAHAEINEAGREVVGSAEAGVDAASVSEEFRADHPFLFCIKHIATNAVLFFGRCVSP

SEQ ID NO: 47 - protein, 802 aa, synthetic construct
  source 1..802: note = LAMP[OVA]
MAAPGSARRPLLLLLLLLLLGLMHCASAAMFMVKNGNGTACIMANFSAAFSVNYDTKSGPKNMTFDLPSDATVVLNRSSCGKENTSDPSLVIAFGRGHTLTLNFTRNATRYSVQLMSFVYNLSDTHLFPNASSKEIKTVESITDIRADIDKKYRCVSGTQVHMNNVTVTLHDATIQAYLSNSSFSRGETRCEQDRPSPTTAPPAPPSPSPSPVPKSPSVDKYNVSGTNGTCLLASMGLQLNLTYERKDNTTVTRLLNINPNKTSASGSCGAHLVTLELHSEGTTVLLFQFGMNASSSRFFLQGIQLNTILPDARDPAFKAANGSLRALQATVGNSYKCNAEEHVRVTKAFSVNIFKVWVQAFKVEGGQFGSVEECLLDENSMGSIGAASMEFCFDVFKELKVHHANENIFYCPIAIMSALAMVYLGAKDSTRTQINKVVRFDKLPGFGDSIEAQCGTSVNVHSSLRDILNQITKPNDVYSFSLASRLYAEERYPILPEYLQCVKELYRGGLEPINFQTAADQARELINSWVESQTNGIIRNVLQPSSVDSQTAMVLVNAIVFKGLWEKTFKDEDTQAMPFRVTEQESKPVQMMYQIGLFRVASMASEKMKILELPFASGTMSMLVLLPDEVSGLEQLESIINFEKLTEWTSSNVMEERKIKVYLPRMKMEEKYNLTSVLMAMGITDVFSSSANLSGISSAESLKISQAVHAAHAEINEAGREVVGSAEAGVDAASVSEEFRADHPFLFCIKHIATNAVLFFGRCVSPLIPIAVGGALAGLVLIVLIAYLVGRKRSHAGYQTI

SEQ ID NO: 48 - DNA, 1866 bp, synthetic construct
  source 1..1866: mol_type = other DNA; note = VAMP7-OVA
atggccatcctgttcgccgtggtggctagaggcacaaccattctggccaagcacgcttggtgcggcggcaactttctggaagtgaccgagcagatcctggccaagattcccagcgagaacaacaagctgacctacagccacggcaactacctgttccactacatctgccaggaccggatcgtgtacctgtgcatcaccgacgacgacttcgagcggagcagagccttcaacttcctgaacgagatcaagaagcggttccagaccacctacggcagcagagcacaaacagccctgccttacgccatgaacagcgagttcagctctgtgctggccgctcagctgaagcaccactccgagaacaaaggcctggacaaagtgatggaaacacaggcccaggtggacgagctgaagggcatcatggtccgaaacatcgacctggtggcccagagaggcgagagactggaactgctgatcgacaagaccgagaacctggtggacagcagcgtgaccttcaagaccaccagcagaaacctggccagagccatgtgcatgaagaacctgaagctgacgatcatcatcattatcgtgtccatcgtgttcatctacatcatcgtgtccccactgtgtggcggcttcacctggcctagctgtgtgaagaaatctggcggcggaggatctggcggaggtggaagcggaggcggaggaagtggatctattggagccgccagcatggaattttgcttcgacgtgttcaaagaactgaaggtgcaccacgccaacgagaacatcttctactgccctatcgccatcatgagcgccctggctatggtgtatctgggcgccaaggacagcacccggacacagatcaacaaggtcgtcagattcgacaagctgcccggcttcggcgattctatcgaagcccagtgtggcaccagcgtgaacgtgcacagcagcctgagagacatcctgaatcagatcaccaagcctaacgacgtgtactccttcagcctggccagcagactgtacgccgaggaaagataccccatcctgcctgagtacctgcagtgcgtgaaagagctgtacagaggcggcctggaacctatcaacttccagacagccgccgaccaggccagagagctgatcaattcttgggtcgagagccagaccaacggcatcatcagaaacgtgctgcagcccagctccgtggattctcagacagccatggtgctggtcaacgccattgtgtttaaaggcctgtgggagaaaaccttcaaggacgaggacacccaggccatgcctttcagagtgacagagcaagagtccaagcctgtgcagatgatgtaccagatcggcctgtttagagtggcctccatggcctccgagaagatgaagatcctcgagctgcctttcgccagcggcaccatgtctatgctggtgctgctgcctgatgaggtgtccggactggaacagctcgagagcatcatcaacttcgagaagctgaccgagtggaccagcagcaacgtgatggaagaacggaagatcaaggtgtacctgcctcggatgaagatggaagagaagtacaacctgaccagcgtgctgatggctatgggcatcacagacgtgttctccagcagcgccaatctgagcggcatcagctctgccgagagcctgaagatttctcaggccgtgcatgctgcccacgccgagattaacgaagccggcagagaagttgtgggatctgccgaagcaggcgtggacgctgcttctgtgtctgaggaattccgggccgaccatccttttctgttctgcatcaagcacattgccaccaacgccgtgctgttctttggcagatgcgtgtccccttga

SEQ ID NO: 49 - DNA, 1974 bp, synthetic construct
  source 1..1974: mol_type = other DNA; note = GOSR2-OVA
atggatcctctgttccagcagacccacaaacaggtgcacgagatccagagctgcatgggcagactggaaaccgccgataagcagagcgtgcacatcgtggaaaatgagatccaggccagcatcgaccagatcttcagcaggctggaacggctggaaatcctgagcagcaaagagcctcctaacaagcggcagaacgcccggctgagagtggaccagctgaagtacgatgtccagcacctccagacagccctgcggaactttcagcacagaaggcacgccagagagcagcaagaacggcagagagaggaactgctgagccggaccttcaccaccaacgacagcgacaccaccattcctatggacgagagcctgcagttcaacagcagcctgcagaaagtgcacaacggcatggacgacctgatcctggacggccacaatatcctggatggcctgagaacccagcggctgacactgaagggcacccagaagaagatcctggatatcgccaacatgctgggcctgagcaacaccgtgatgcggctgattgagaagcgggccttccaggacaagtacttcatgatcgagacacggtcccaccacgtggcccagaatggacctgaactgctgtccagcagagatcctcctgccagcgcctctagatctgccggcatcatcggcatgagccaccatcctgacctgcagatccctttcgagctgagactgggcttcgagctgtggttctatcagctgctggccgtgatcagcgaccaaggcggcggaggatctggcggaggtggaagcggaggcggaggaagtggatctattggagccgccagcatggaattttgcttcgacgtgttcaaagaactgaaggtgcaccacgccaacgagaacatcttctactgccctatcgccatcatgagcgccctggctatggtgtatctgggcgccaaggacagcacccggacacagatcaacaaggtcgtcagattcgacaagctgcccggcttcggcgattctatcgaagcccagtgtggcaccagcgtgaacgtgcacagcagcctgagagacatcctgaatcagatcaccaagcctaacgacgtgtactccttcagcctggccagcagactgtacgccgaggaaagataccccatcctgcctgagtacctgcagtgcgtgaaagagctgtacagaggcggcctggaacctatcaacttccagacagccgccgaccaggccagagagctgatcaattcttgggtcgagagccagaccaacggcatcatcagaaacgtgctgcagcccagctccgtggattctcagacagccatggtgctggtcaacgccattgtgtttaaaggcctgtgggagaaaaccttcaaggacgaggacacccaggccatgcctttcagagtgacagagcaagagtccaagcctgtgcagatgatgtaccagatcggcctgtttagagtggcctccatggcctccgagaagatgaagatcctcgagctgcctttcgccagcggcaccatgtctatgctggtgctgctgcctgatgaggtgtccggactggaacagctcgagagcatcatcaacttcgagaagctgaccgagtggaccagcagcaacgtgatggaagaacggaagatcaaggtgtacctgcctcggatgaagatggaagagaagtacaacctgaccagcgtgctgatggctatgggcatcacagacgtgttctccagcagcgccaatctgagcggcatcagctctgccgagagcctgaagatttctcaggccgtgcatgctgcccacgccgagattaacgaagccggcagagaagttgtgggatctgccgaagcaggcgtggacgctgcttctgtgtctgaggaattccgggccgaccatccttttctgttctgcatcaagcacattgccaccaacgccgtgctgttctttggcagatgcgtgtccccttga

SEQ ID NO: 50 - DNA, 1950 bp, synthetic construct
  source 1..1950: mol_type = other DNA; note = STX10-OVA
atgagcctggaagatcccttctttgtcgtgcgcggcgaggtgcagaaagccgtgaatactgccagaggcctgtaccagcgttggtgcgagctgctgcaagaatctgccgctgtgggcagagaggaactggactggaccaccaacgagctgagaaacggcctgagatccatcgagtgggacctcgaggacctggaagagacaatcggcatcgtggaagccaatcctggcaagttcaaactgcctgccggcgacctgcaagagcggaaggtgttcgtggaacggatgcgggaagccgtgcaagagatgaaggaccacatggtgtctccaaccgccgtggccttcctggaacggaacaacagagagatcctggccggaaagcctgccgctcagaagtctcctagcgatctgctggatgcctctgccgtgtctgccacaagccggtacattgaggaacagcaggccacacagcagctgatcatggacgagcaggaccagcagctggaaatggtgtctggcagcatccaggtgctgaagcacatgagcggaagagtgggcgaagaactggatgagcagggcatcatgctggacgccttcgctcaagagatggatcacacccagagccggatggacggcgtgctgagaaagctggccaaagtgtcccacatgaccagcgaccgtagacagtggtgcgccattgctgtgcttgtgggagtgctgctgctggtgctgatcctgctgtttagccttggcggcggaggatctggcggaggtggaagcggaggcggaggaagtggatctattggagccgccagcatggaattttgcttcgacgtgttcaaagaactgaaggtgcaccacgccaacgagaacatcttctactgccctatcgccatcatgagcgccctggctatggtgtatctgggcgccaaggacagcacccggacacagatcaacaaggtcgtcagattcgacaagctgcccggcttcggcgattctatcgaagcccagtgtggcaccagcgtgaacgtgcacagcagcctgagagacatcctgaatcagatcaccaagcctaacgacgtgtactccttcagcctggccagcagactgtacgccgaggaaagataccccatcctgcctgagtacctgcagtgcgtgaaagagctgtacagaggcggcctggaacctatcaacttccagacagccgccgaccaggccagagagctgatcaattcttgggtcgagagccagaccaacggcatcatcagaaacgtgctgcagcccagctccgtggattctcagacagccatggtgctggtcaacgccattgtgtttaaaggcctgtgggagaaaaccttcaaggacgaggacacccaggccatgcctttcagagtgacagagcaagagtccaagcctgtgcagatgatgtaccagatcggcctgtttagagtggcctccatggcctccgagaagatgaagatcctcgagctgcctttcgccagcggcaccatgtctatgctggtgctgctgcctgatgaggtgtccggactggaacagctcgagagcatcatcaacttcgagaagctgaccgagtggaccagcagcaacgtgatggaagaacggaagatcaaggtgtacctgcctcggatgaagatggaagagaagtacaacctgaccagcgtgctgatggctatgggcatcacagacgtgttctccagcagcgccaatctgagcggcatcagctctgccgagagcctgaagatttctcaggccgtgcatgctgcccacgccgagattaacgaagccggcagagaagttgtgggatctgccgaagcaggcgtggacgctgcttctgtgtctgaggaattccgggccgaccatccttttctgttctgcatcaagcacattgccaccaacgccgtgctgttctttggcagatgcgtgtccccttga

SEQ ID NO: 51 - DNA, 2208 bp, synthetic construct
  source 1..2208: mol_type = other DNA; note = STX18-OVA
atggccgtggatatcaccctgctgtttcgggccagcgtgaaaacagtgaaaacccggaacaaggccctgggcgttgcagttggaggcggagttgatggcagcagggatgagctgttcagaagaagccccagacctaagggcgacttcagcagcagagcccgggaagtgatcagccacatcggcaagctgagagacttcctgctggaacaccggaaggactacatcaacgcctacagccacaccatgagcgagtacggcagaatgaccgacaccgagagggaccagatcgaccaggatgcccagatcttcatgcggacctgtagcgaggccatccagcagctgagaacagaggcccacaaagagatccacagccagcaagtgaaagaacacagaaccgccgtgctggacttcatcgaggactacctgaagagagtgtgcaagctgtactccgagcagcgggccatcagagtgaaaagagtggtggacaagaagcggctgagcaagctggaacccgagcctaacaccaagaccagagagagcaccagctccgagaaagtgtctcagagccccagcaaggacagcgaggaaaatcctgccaccgaggaacggcccgagaagattctggctgagacacagcctgaactcggcacctggggagatggcaagggcgaagatgaactgagccccgaagagattcagatgttcgagcaagagaaccagcggctgatcggcgagatgaacagcctgtttgacgaagtgcggcagatcgagggccgcgtggtggaaatctctcggctgcaagagatcttcaccgagaaggtcctgcagcaagaggccgagatcgacagcatccatcagctggttgtgggcgccaccgagaacatcaaagagggcaacgaggacatcagagaggccatcaagaacaacgccggcttcagagtgtggatcctgttcttcctggtcatgtgcagcttcagcctgctgttcctggattggtacgactctggcggcggaggatctggcggaggtggaagcggaggcggaggaagtggatctattggagccgccagcatggaattttgcttcgacgtgttcaaagaactgaaggtgcaccacgccaacgagaacatcttctactgccctatcgccatcatgagcgccctggctatggtgtatctgggcgccaaggacagcacccggacacagatcaacaaggtcgtcagattcgacaagctgcccggcttcggcgattctatcgaagcccagtgtggcaccagcgtgaacgtgcacagcagcctgagagacatcctgaatcagatcaccaagcctaacgacgtgtactccttcagcctggccagcagactgtacgccgaggaaagataccccatcctgcctgagtacctgcagtgcgtgaaagagctgtacagaggcggcctggaacctatcaacttccagacagccgccgaccaggccagagagctgatcaattcttgggtcgagagccagaccaacggcatcatcagaaacgtgctgcagcccagctccgtggattctcagacagccatggtgctggtcaacgccattgtgtttaaaggcctgtgggagaaaaccttcaaggacgaggacacccaggccatgcctttcagagtgacagagcaagagtccaagcctgtgcagatgatgtaccagatcggcctgtttagagtggcctccatggcctccgagaagatgaagatcctcgagctgcctttcgccagcggcaccatgtctatgctggtgctgctgcctgatgaggtgtccggactggaacagctcgagagcatcatcaacttcgagaagctgaccgagtggaccagcagcaacgtgatggaagaacggaagatcaaggtgtacctgcctcggatgaagatggaagagaagtacaacctgaccagcgtgctgatggctatgggcatcacagacgtgttctccagcagcgccaatctgagcggcatcagctctgccgagagcctgaagatttctcaggccgtgcatgctgcccacgccgagattaacgaagccggcagagaagttgtgggatctgccgaagcaggcgtggacgctgcttctgtgtctgaggaattccgggccgaccatccttttctgttctgcatcaagcacattgccaccaacgccgtgctgttctttggcagatgcgtgtccccttga

SEQ ID NO: 52 - DNA, 2016 bp, synthetic construct
  source 1..2016: mol_type = other DNA; note = BNIP1-OVA
atggctgctcctcaggatgtgcacgtgcggatctgcaatcaagagatcgtgaagttcgacctggaagtgaaggccctgatccaggacatcagagactgtagcggacctctgagcgccctgaccgagctgaacaccaaagtgaaagagaagttccagcagctgcggcaccggatccagcctgtgctgtatcagagagccttcatctggaccgccagcaccttctttttcaaactgacctacagcctgaccgacttcagcagcacccagcacgacttcaacagccctaccacacctgtgaccttcagcgatctggaacagctggccaaagagcaggacaaagagagcgagaaacagctgctgctgcaagaggtggaaaaccacaaaaagcagatgctgagcaaccaggcctcctggcggaaggccaatctgacatgcaagatcgccatcgacaacctggaaaaggccgagctgctccaaggcggcgatctgctgagacagagaaagaccaccaaagagtctctggcccagaccagctccaccatcaccgaatctctgatgggcatcagcagaatgatggcccagcaggtccagcagagcgaggaagccatgcagagcctggtcaccagcagcagaacaatcctggacgccaacgaggaattcaagagcatgagcggcaccatccagctgggcagaaagctgatcaccaagtacaacagaagagagctgaccgacaagctgctgatcttcctggctctggccctgtttctggccaccgtgctgtacatcgtgaagaagcggctgttcccattccttggcggcggaggatctggcggaggtggaagcggaggcggaggaagtggatctattggagccgccagcatggaattttgcttcgacgtgttcaaagaactgaaggtgcaccacgccaacgagaacatcttctactgccctatcgccatcatgagcgccctggctatggtgtatctgggcgccaaggacagcacccggacacagatcaacaaggtcgtcagattcgacaagctgcccggcttcggcgattctatcgaagcccagtgtggcaccagcgtgaacgtgcacagcagcctgagagacatcctgaatcagatcaccaagcctaacgacgtgtactccttcagcctggccagcagactgtacgccgaggaaagataccccatcctgcctgagtacctgcagtgcgtgaaagagctgtacagaggcggcctggaacctatcaacttccagacagccgccgaccaggccagagagctgatcaattcttgggtcgagagccagaccaacggcatcatcagaaacgtgctgcagcccagctccgtggattctcagacagccatggtgctggtcaacgccattgtgtttaaaggcctgtgggagaaaaccttcaaggacgaggacacccaggccatgcctttcagagtgacagagcaagagtccaagcctgtgcagatgatgtaccagatcggcctgtttagagtggcctccatggcctccgagaagatgaagatcctcgagctgcctttcgccagcggcaccatgtctatgctggtgctgctgcctgatgaggtgtccggactggaacagctcgagagcatcatcaacttcgagaagctgaccgagtggaccagcagcaacgtgatggaagaacggaagatcaaggtgtacctgcctcggatgaagatggaagagaagtacaacctgaccagcgtgctgatggctatgggcatcacagacgtgttctccagcagcgccaatctgagcggcatcagctctgccgagagcctgaagatttctcaggccgtgcatgctgcccacgccgagattaacgaagccggcagagaagttgtgggatctgccgaagcaggcgtggacgctgcttctgtgtctgaggaattccgggccgaccatccttttctgttctgcatcaagcacattgccaccaacgccgtgctgttctttggcagatgcgtgtccccttga

SEQ ID NO: 53 - DNA, 1986 bp, synthetic construct
  source 1..1986: mol_type = other DNA; note = STX7-OVA
atgagctacacacctggcgttggcggagatcctgctcagctggcccagagaatcagcagcaacatccagaaaatcacccagtgcagcgtggaaatccagcggaccctgaatcagctgggcacccctcaggatagccctgagctgagacagcagctgcagcagaagcagcagtacaccaaccagctggccaaagagacagacaagtacatcaaagagttcggcagcctgcctaccacacctagcgagcagagacagcggaagatccagaaagacagactggtggccgagttcaccaccagcctgaccaacttccagaaggtgcagaggcaggccgctgagcgcgagaaagaatttgtggccagagtgcgggccagcagcagagtgtcaggatcctttccagaggacagctccaaagagcggaacctggtttcctgggagagccagacacagcctcaggtgcaggtccaggacgaggaaatcaccgaggacgacctgagactgatccacgagagagagtccagcatccggcagctggaagccgacatcatggacatcaacgagatcttcaaggacctgggcatgatgattcacgagcagggcgacgtgatcgacagcatcgaggccaacgtggaaaacgccgaagtgcatgtgcagcaggccaaccagcagctgtctagagccgccgactaccagcgcaagagcagaaagaccctgtgcatcatcatcctgatcctggtcatcggcgtggccatcatctccctgatcatctggggcctgaaccatggcggcggaggatctggcggaggtggaagcggaggcggaggaagtggatctattggagccgccagcatggaattttgcttcgacgtgttcaaagaactgaaggtgcaccacgccaacgagaacatcttctactgccctatcgccatcatgagcgccctggctatggtgtatctgggcgccaaggacagcacccggacacagatcaacaaggtcgtcagattcgacaagctgcccggcttcggcgattctatcgaagcccagtgtggcaccagcgtgaacgtgcacagcagcctgagagacatcctgaatcagatcaccaagcctaacgacgtgtactccttcagcctggccagcagactgtacgccgaggaaagataccccatcctgcctgagtacctgcagtgcgtgaaagagctgtacagaggcggcctggaacctatcaacttccagacagccgccgaccaggccagagagctgatcaattcttgggtcgagagccagaccaacggcatcatcagaaacgtgctgcagcccagctccgtggattctcagacagccatggtgctggtcaacgccattgtgtttaaaggcctgtgggagaaaaccttcaaggacgaggacacccaggccatgcctttcagagtgacagagcaagagtccaagcctgtgcagatgatgtaccagatcggcctgtttagagtggcctccatggcctccgagaagatgaagatcctcgagctgcctttcgccagcggcaccatgtctatgctggtgctgctgcctgatgaggtgtccggactggaacagctcgagagcatcatcaacttcgagaagctgaccgagtggaccagcagcaacgtgatggaagaacggaagatcaaggtgtacctgcctcggatgaagatggaagagaagtacaacctgaccagcgtgctgatggctatgggcatcacagacgtgttctccagcagcgccaatctgagcggcatcagctctgccgagagcctgaagatttctcaggccgtgcatgctgcccacgccgagattaacgaagccggcagagaagttgtgggatctgccgaagcaggcgtggacgctgcttctgtgtctgaggaattccgggccgaccatccttttctgttctgcatcaagcacattgccaccaacgccgtgctgttctttggcagatgcgtgtccccttga

SEQ ID NO: 54 - DNA, 1875 bp, synthetic construct
  source 1..1875: mol_type = other DNA; note = VTI1A-OVA
atgagcagcgacttcgagggctacgagcaggattttgccgtgctgaccgccgagatcaccagcaagattgccagagtgcccagactgcctcctgacgagaagaaacagatggtggccaacgtggaaaagcagctggaagaggccaaagaactgctggaacagatggacctggaagtgcgcgagatccctccacagagcagaggcatgtacagcaaccggatgcggagctacaagcaagagatgggcaagctggaaaccgacttcaagcggagcagaatcgcctacagcgacgaagtgcggaatgagctgctgggcgacgatggcaacagcagcgagaaccagctgatcaagctgcgggaagagagagcccatctgctggacaacaccgagcggctggaaagaagcagcagaaggctggaagccggctatcagatcgccgtggaaactgagcagatcggccaagagatgctggaaaacctgagccacgacagagagaagatccagcgggccagagagcggctgagagagacagacgccaatctgggcaagagcagcaggattctgaccggcatgctgcggcggatcatccagaataggatcctgctggtcatcctgggcatcatcgtggtcatcaccatcctgatggccattaccttcagcgtgcggcggcatggcggcggaggatctggcggaggtggaagcggaggcggaggaagtggatctattggagccgccagcatggaattttgcttcgacgtgttcaaagaactgaaggtgcaccacgccaacgagaacatcttctactgccctatcgccatcatgagcgccctggctatggtgtatctgggcgccaaggacagcacccggacacagatcaacaaggtcgtcagattcgacaagctgcccggcttcggcgattctatcgaagcccagtgtggcaccagcgtgaacgtgcacagcagcctgagagacatcctgaatcagatcaccaagcctaacgacgtgtactccttcagcctggccagcagactgtacgccgaggaaagataccccatcctgcctgagtacctgcagtgcgtgaaagagctgtacagaggcggcctggaacctatcaacttccagacagccgccgaccaggccagagagctgatcaattcttgggtcgagagccagaccaacggcatcatcagaaacgtgctgcagcccagctccgtggattctcagacagccatggtgctggtcaacgccattgtgtttaaaggcctgtgggagaaaaccttcaaggacgaggacacccaggccatgcctttcagagtgacagagcaagagtccaagcctgtgcagatgatgtaccagatcggcctgtttagagtggcctccatggcctccgagaagatgaagatcctcgagctgcctttcgccagcggcaccatgtctatgctggtgctgctgcctgatgaggtgtccggactggaacagctcgagagcatcatcaacttcgagaagctgaccgagtggaccagcagcaacgtgatggaagaacggaagatcaaggtgtacctgcctcggatgaagatggaagagaagtacaacctgaccagcgtgctgatggctatgggcatcacagacgtgttctccagcagcgccaatctgagcggcatcagctctgccgagagcctgaagatttctcaggccgtgcatgctgcccacgccgagattaacgaagccggcagagaagttgtgggatctgccgaagcaggcgtggacgctgcttctgtgtctgaggaattccgggccgaccatccttttctgttctgcatcaagcacattgccaccaacgccgtgctgttctttggcagatgcgtgtccccttga

SEQ ID NO: 55 - DNA, 2178 bp, synthetic construct
  source 1..2178: mol_type = other DNA; note = STX16-OVA
atggccaccagaaggctgacagacgctttcctgctgctgcggaacaacagcatccagaacagacagctgctggccgaacaggtgtccagccacatcacatctagccctctgcacagcagatctatcgccgccgagctggatgagctggccgatgatagaatggccctggtgtccggcatctctctggatcctgaagccgccatcggcgtgaccaaacggcctcctcctaaatgggttgacggcgtggacgagatccagtacgacgtgggcagaatcaagcagaagatgaaggaactggccagcctgcacgacaagcacctgaacagacccacactggacgacagcagcgaggaagaacacgccatcgagatcaccacacaagagatcacccagctgttccaccggtgccagagagctgttcaggccctgccttctagagccagagcctgctctgagcaagagggcagactgctgggaaacgtggtggcttctctggctcaggctctgcaagagctgagcaccagctttagacacgcccagagcggctacctgaagcggatgaagaaccgggaagagagatcccagcacttcttcgacaccagcgtgcccctgatggacgacggcgacgataataccctgtaccacagaggcttcaccgaggaccagctcgtgctggttgagcagaacaccctgatggtggaagaacgcgagcgcgagatcagacagatcgtgcagagcatcagcgacctgaacgagatcttcagagatctgggcgccatgatcgtggaacagggcaccgtgctggaccggatcgactacaatgtggaacagagctgcatcaagaccgaggacggactgaagcagctgcacaaagccgagcagtaccagaaaaagaatcggaagatgctggtcatcctgatcctgttcgtgatcatcatcgtgctgatcgtggtgctcgtgggcgtgaagtctagaggcggcggaggatctggcggaggtggaagcggaggcggaggaagtggatctattggagccgccagcatggaattttgcttcgacgtgttcaaagaactgaaggtgcaccacgccaacgagaacatcttctactgccctatcgccatcatgagcgccctggctatggtgtatctgggcgccaaggacagcacccggacacagatcaacaaggtcgtcagattcgacaagctgcccggcttcggcgattctatcgaagcccagtgtggcaccagcgtgaacgtgcacagcagcctgagagacatcctgaatcagatcaccaagcctaacgacgtgtactccttcagcctggccagcagactgtacgccgaggaaagataccccatcctgcctgagtacctgcagtgcgtgaaagagctgtacagaggcggcctggaacctatcaacttccagacagccgccgaccaggccagagagctgatcaattcttgggtcgagagccagaccaacggcatcatcagaaacgtgctgcagcccagctccgtggattctcagacagccatggtgctggtcaacgccattgtgtttaaaggcctgtgggagaaaaccttcaaggacgaggacacccaggccatgcctttcagagtgacagagcaagagtccaagcctgtgcagatgatgtaccagatcggcctgtttagagtggcctccatggcctccgagaagatgaagatcctcgagctgcctttcgccagcggcaccatgtctatgctggtgctgctgcctgatgaggtgtccggactggaacagctcgagagcatcatcaacttcgagaagctgaccgagtggaccagcagcaacgtgatggaagaacggaagatcaaggtgtacctgcctcggatgaagatggaagagaagtacaacctgaccagcgtgctgatggctatgggcatcacagacgtgttctccagcagcgccaatctgagcggcatcagctctgccgagagcctgaagatttctcaggccgtgcatgctgcccacgccgagattaacgaagccggcagagaagttgtgggatctgccgaagcaggcgtggacgctgcttctgtgtctgaggaattccgggccgaccatccttttctgttctgcatcaagcacattgccaccaacgccgtgctgttctttggcagatgcgtgtccccttga

SEQ ID NO: 56 - DNA, 2268 bp, synthetic construct
  source 1..2268: mol_type = other DNA; note = STX5-OVA
atgattccccggaagagatacggcagcaagaacaccgatcagggcgtgtacctgggcctgagcaaaacacaggtgctgtctccagccacagccggcagctctagctctgatattgctcccctgcctcctcctgtgacactggttcctccaccacctgacaccatgagctgcagagacagaacccaagagttcctgagcgcctgcaagagcctgcagaccagacagaatggcatccagaccaacaagcccgctctgagagccgtgcggcagagaagcgagtttaccctgatggccaagcggatcggcaaggacctgagcaacaccttcgccaagctggaaaagctgaccatcctggccaagagaaagagcctgttcgacgacaaggccgtggaaatcgaggaactgacctacatcatcaagcaggacatcaacagcctgaacaagcagatcgcccagctgcaggacttcgtcagagccaagggaagccagagcggcagacacctccagacacacagcaacaccatcgtggtgtccctgcagagcaagctggcctccatgagcaacgacttcaagagcgtgctggaagtgcggaccgagaacctgaagcagcagcggtctagaagagagcagttcagcagagcccctgtgtctgctctgcccctggctcctaatcatcttggaggcggagctgtggtgctgggagccgaatctcacgcctctaaggacgtggccatcgacatgatggacagcagaaccagccagcagctgcaactgatcgacgagcaggacagctacatccagagcagagccgacaccatgcagaacatcgagagcacaatcgtggaactgggcagcatctttcagcagctggcccacatggtcaaagagcaagaggaaaccatccagcgcatcgacgagaatgtgctgggcgctcagctggatgtggaagccgctcactctgagatcctgaagtactttcagagcgtgaccagcaaccggtggctgatggtcaagatcttcctgatcctgatcgtgttctttattatcttcgtcgtgttcctggctggcggcggaggatctggcggaggtggaagcggaggcggaggaagtggatctattggagccgccagcatggaattttgcttcgacgtgttcaaagaactgaaggtgcaccacgccaacgagaacatcttctactgccctatcgccatcatgagcgccctggctatggtgtatctgggcgccaaggacagcacccggacacagatcaacaaggtcgtcagattcgacaagctgcccggcttcggcgattctatcgaagcccagtgtggcaccagcgtgaacgtgcacagcagcctgagagacatcctgaatcagatcaccaagcctaacgacgtgtactccttcagcctggccagcagactgtacgccgaggaaagataccccatcctgcctgagtacctgcagtgcgtgaaagagctgtacagaggcggcctggaacctatcaacttccagacagccgccgaccaggccagagagctgatcaattcttgggtcgagagccagaccaacggcatcatcagaaacgtgctgcagcccagctccgtggattctcagacagccatggtgctggtcaacgccattgtgtttaaaggcctgtgggagaaaaccttcaaggacgaggacacccaggccatgcctttcagagtgacagagcaagagtccaagcctgtgcagatgatgtaccagatcggcctgtttagagtggcctccatggcctccgagaagatgaagatcctcgagctgcctttcgccagcggcaccatgtctatgctggtgctgctgcctgatgaggtgtccggactggaacagctcgagagcatcatcaacttcgagaagctgaccgagtggaccagcagcaacgtgatggaagaacggaagatcaaggtgtacctgcctcggatgaagatggaagagaagtacaacctgaccagcgtgctgatggctatgggcatcacagacgtgttctccagcagcgccaatctgagcggcatcagctctgccgagagcctgaagatttctcaggccgtgcatgctgcccacgccgagattaacgaagccggcagagaagttgtgggatctgccgaagcaggcgtggacgctgcttctgtgtctgaggaattccgggccgaccatccttttctgttctgcatcaagcacattgccaccaacgccgtgctgttctttggcagatgcgtgtccccttga

SEQ ID NO: 57 - DNA, 1968 bp, synthetic construct
  source 1..1968: mol_type = other DNA; note = STX6-OVA
atgagcatggaagatccattcttcgtggtcaagggcgaagtgcagaaagccgtgaacacagcccagggcctgttccagagatggacagagctgctgcaggaccctagcaccgccaccagagaggaaatcgactggaccaccaacgagctgcggaacaacctgagatccatcgagtgggacctcgaggacctggacgagacaatcagcatcgtggaagccaatcctcggaagttcaacctggacgccaccgagctgagcatcagaaaggccttcatcaccagcaccagacaggtcgtgcgggacatgaaggaccagatgagcacaagctctgtgcaggctctggccgagcggaagaatagacaggctctgctgggcgatagcggcagccagaattggagcaccggcaccacagataagtacggcagactggatagagagctgcagcgggccaacagccacttcatcgaagaacagcaggcccagcagcagctgatcgtcgagcagcaggatgagcagctggaactggtgtctggctctatcggcgtgctgaagaacatgagccagagaatcggcggcgaactggaagaacaggccgtgatgctggaagatttcagccacgagctggaaagcacccagagcaggctggacaacgtgatgaagaagctggccaaggtttcccacatgaccagcgaccgtagacagtggtgcgccattgccatcctgtttgccgtgctgctggtggtgctgatcctgttcctggtgcttggcggcggaggatctggcggaggtggaagcggaggcggaggaagtggatctattggagccgccagcatggaattttgcttcgacgtgttcaaagaactgaaggtgcaccacgccaacgagaacatcttctactgccctatcgccatcatgagcgccctggctatggtgtatctgggcgccaaggacagcacccggacacagatcaacaaggtcgtcagattcgacaagctgcccggcttcggcgattctatcgaagcccagtgtggcaccagcgtgaacgtgcacagcagcctgagagacatcctgaatcagatcaccaagcctaacgacgtgtactccttcagcctggccagcagactgtacgccgaggaaagataccccatcctgcctgagtacctgcagtgcgtgaaagagctgtacagaggcggcctggaacctatcaacttccagacagccgccgaccaggccagagagctgatcaattcttgggtcgagagccagaccaacggcatcatcagaaacgtgctgcagcccagctccgtggattctcagacagccatggtgctggtcaacgccattgtgtttaaaggcctgtgggagaaaaccttcaaggacgaggacacccaggccatgcctttcagagtgacagagcaagagtccaagcctgtgcagatgatgtaccagatcggcctgtttagagtggcctccatggcctccgagaagatgaagatcctcgagctgcctttcgccagcggcaccatgtctatgctggtgctgctgcctgatgaggtgtccggactggaacagctcgagagcatcatcaacttcgagaagctgaccgagtggaccagcagcaacgtgatggaagaacggaagatcaaggtgtacctgcctcggatgaagatggaagagaagtacaacctgaccagcgtgctgatggctatgggcatcacagacgtgttctccagcagcgccaatctgagcggcatcagctctgccgagagcctgaagatttctcaggccgtgcatgctgcccacgccgagattaacgaagccggcagagaagttgtgggatctgccgaagcaggcgtggacgctgcttctgtgtctgaggaattccgggccgaccatccttttctgttctgcatcaagcacattgccaccaacgccgtgctgttctttggcagatgcgtgtccccttga

SEQ ID NO: 58 - DNA, 1911 bp, synthetic construct
  source 1..1911: mol_type = other DNA; note = STX8-OVA
atggctcccgatccatggttcagcacctacgacagcacctgtcagatcgcccaagagatcgccgagaagatccagcagcggaaccagtacgagcggaagggcgagaaagcccctaagctgaccgtgaccattagagccctgctgcagaacctgaaagagaagatcgccctgctgaaggatctgctgctgagagccgtgtctacccaccagatcacacagctggaaggcgaccgcagacagaacctgctggatgacctggtcaccagagagagactgctgctggcctccttcaagaacgaaggcgccgagcctgacctgatcagatccagcctgatgagcgaggaagccaagagaggcgcccctaatccttggctgttcgaggaacccgaggaaaccagaggcctgggcttcgacgagatcagacagcagcagcaaaagatcatccaagagcaggacgccggcctggatgccctgtctagcatcatcagccggcagaaacagatgggccaagagattggcaacgagctggacgagcagaacgagatcatcgacgacctggccaacctggtggaaaacaccgacgagaagctgcggaacgagactcggagagtgaacatggtggaccggaagtctgccagctgcgggatgatcatggttatcctgttgctgctggtggccatcgtggtggtggctgtgtggcctacaaatggcggcggaggatctggcggaggtggaagcggaggcggaggaagtggatctattggagccgccagcatggaattttgcttcgacgtgttcaaagaactgaaggtgcaccacgccaacgagaacatcttctactgccctatcgccatcatgagcgccctggctatggtgtatctgggcgccaaggacagcacccggacacagatcaacaaggtcgtcagattcgacaagctgcccggcttcggcgattctatcgaagcccagtgtggcaccagcgtgaacgtgcacagcagcctgagagacatcctgaatcagatcaccaagcctaacgacgtgtactccttcagcctggccagcagactgtacgccgaggaaagataccccatcctgcctgagtacctgcagtgcgtgaaagagctgtacagaggcggcctggaacctatcaacttccagacagccgccgaccaggccagagagctgatcaattcttgggtcgagagccagaccaacggcatcatcagaaacgtgctgcagcccagctccgtggattctcagacagccatggtgctggtcaacgccattgtgtttaaaggcctgtgggagaaaaccttcaaggacgaggacacccaggccatgcctttcagagtgacagagcaagagtccaagcctgtgcagatgatgtaccagatcggcctgtttagagtggcctccatggcctccgagaagatgaagatcctcgagctgcctttcgccagcggcaccatgtctatgctggtgctgctgcctgatgaggtgtccggactggaacagctcgagagcatcatcaacttcgagaagctgaccgagtggaccagcagcaacgtgatggaagaacggaagatcaaggtgtacctgcctcggatgaagatggaagagaagtacaacctgaccagcgtgctgatggctatgggcatcacagacgtgttctccagcagcgccaatctgagcggcatcagctctgccgagagcctgaagatttctcaggccgtgcatgctgcccacgccgagattaacgaagccggcagagaagttgtgggatctgccgaagcaggcgtggacgctgcttctgtgtctgaggaattccgggccgaccatccttttctgttctgcatcaagcacattgccaccaacgccgtgctgttctttggcagatgcgtgtccccttga

SEQ ID NO: 59 - DNA, 2031 bp, synthetic construct
  source 1..2031: mol_type = other DNA; note = STX12-OVA
atgagctacggccctctggacatgtacagaaaccccggaccttctggcccacagctgagagacttcagcagcatcatccagacctgcagcggcaacatccagagaatcagccaggccaccgctcagatcaagaacctgatgagccagctgggcaccaagcaggacagcagcaagctgcaagagaacctgcagcagctccagcacagcaccaaccagctggccaaagagacaaacgagctgctgaaagagctgggcagcctgcctctgcctctgagcacatctgaacagcggcagcagcggctgcagaaagaacggctgatgaacgacttcagcgccgctctgaacaacttccaggccgtgcagagaagagtgtccgagaaagagaaagagtctatcgccagagccagagccggcagcagactgtctgccgaggaaagacagcgggaagaacagctggtgtccttcgacagccacgaggaatggaaccagatgcagagccaagaggacgaggtggccatcaccgagcaggacctggaactgatcaaagagagagagacagccatccggcagctggaagccgacatcctggatgtgaaccagatcttcaaggacctggccatgatgatccacgaccagggcgacctgatcgacagcatcgaggccaatgtggaaagcagcgaggtgcacgtggaacgggctacagaacaactgcagagagccgcctactaccagaagaaaagccggaagaaaatgtgcatcctggtgctggtcctgagcgtgatcatcctgatcctgggcctgatcatctggctggtgtacaagaccaaaggcggcggaggatctggcggaggtggaagcggaggcggaggaagtggatctattggagccgccagcatggaattttgcttcgacgtgttcaaagaactgaaggtgcaccacgccaacgagaacatcttctactgccctatcgccatcatgagcgccctggctatggtgtatctgggcgccaaggacagcacccggacacagatcaacaaggtcgtcagattcgacaagctgcccggcttcggcgattctatcgaagcccagtgtggcaccagcgtgaacgtgcacagcagcctgagagacatcctgaatcagatcaccaagcctaacgacgtgtactccttcagcctggccagcagactgtacgccgaggaaagataccccatcctgcctgagtacctgcagtgcgtgaaagagctgtacagaggcggcctggaacctatcaacttccagacagccgccgaccaggccagagagctgatcaattcttgggtcgagagccagaccaacggcatcatcagaaacgtgctgcagcccagctccgtggattctcagacagccatggtgctggtcaacgccattgtgtttaaaggcctgtgggagaaaaccttcaaggacgaggacacccaggccatgcctttcagagtgacagagcaagagtccaagcctgtgcagatgatgtaccagatcggcctgtttagagtggcctccatggcctccgagaagatgaagatcctcgagctgcctttcgccagcggcaccatgtctatgctggtgctgctgcctgatgaggtgtccggactggaacagctcgagagcatcatcaacttcgagaagctgaccgagtggaccagcagcaacgtgatggaagaacggaagatcaaggtgtacctgcctcggatgaagatggaagagaagtacaacctgaccagcgtgctgatggctatgggcatcacagacgtgttctccagcagcgccaatctgagcggcatcagctctgccgagagcctgaagatttctcaggccgtgcatgctgcccacgccgagattaacgaagccggcagagaagttgtgggatctgccgaagcaggcgtggacgctgcttctgtgtctgaggaattccgggccgaccatccttttctgttctgcatcaagcacattgccaccaacgccgtgctgttctttggcagatgcgtgtccccttga

SEQ ID NO: 60 - DNA, 1503 bp, synthetic construct
  source 1..1503: mol_type = other DNA; note = VAMP3-OVA
atgagcacaggacctacagccgccacaggcagcaatagaaggctgcagcagacccagaaccaggtggacgaggtggtggacatcatgagagtgaacgtggacaaggtgctggaacgggaccagaagctgagcgagctggacgatagagccgatgctctgcaagctggcgcctctcagtttgagacatctgccgccaagctgaagcggaagtactggtggaagaactgcaagatgtgggccatcggcatcaccgtgctggtcatctttatcatcatcattatcgtgtgggtcgtgtcctctggcggcggaggatctggcggaggtggaagcggaggcggaggaagtggatctattggagccgccagcatggaattttgcttcgacgtgttcaaagaactgaaggtgcaccacgccaacgagaacatcttctactgccctatcgccatcatgagcgccctggctatggtgtatctgggcgccaaggacagcacccggacacagatcaacaaggtcgtcagattcgacaagctgcccggcttcggcgattctatcgaagcccagtgtggcaccagcgtgaacgtgcacagcagcctgagagacatcctgaatcagatcaccaagcctaacgacgtgtactccttcagcctggccagcagactgtacgccgaggaaagataccccatcctgcctgagtacctgcagtgcgtgaaagagctgtacagaggcggcctggaacctatcaacttccagacagccgccgaccaggccagagagctgatcaattcttgggtcgagagccagaccaacggcatcatcagaaacgtgctgcagcccagctccgtggattctcagacagccatggtgctggtcaacgccattgtgtttaaaggcctgtgggagaaaaccttcaaggacgaggacacccaggccatgcctttcagagtgacagagcaagagtccaagcctgtgcagatgatgtaccagatcggcctgtttagagtggcctccatggcctccgagaagatgaagatcctcgagctgcctttcgccagcggcaccatgtctatgctggtgctgctgcctgatgaggtgtccggactggaacagctcgagagcatcatcaacttcgagaagctgaccgagtggaccagcagcaacgtgatggaagaacggaagatcaaggtgtacctgcctcggatgaagatggaagagaagtacaacctgaccagcgtgctgatggctatgggcatcacagacgtgttctccagcagcgccaatctgagcggcatcagctctgccgagagcctgaagatttctcaggccgtgcatgctgcccacgccgagattaacgaagccggcagagaagttgtgggatctgccgaagcaggcgtggacgctgcttctgtgtctgaggaattccgggccgaccatccttttctgttctgcatcaagcacattgccaccaacgccgtgctgttctttggcagatgcgtgtccccttga

SEQ ID NO: 61 - DNA, 1626 bp, synthetic construct
  source 1..1626: mol_type = other DNA; note = VAMP4-OVA
atgcctccaaagttcaagcggcacctgaacgacgacgatgtgaccggctctgtgaagtccgagcggagaaacctgctggaagatgacagcgacgaggaagaggacttcttcctgcggggaccttctggccctagattcggccccagaaacgacaagatcaagcacgtgcagaaccaggtggacgaagtgatcgacgtgatgcaagagaacatcaccaaagtcatcgagcggggcgagagactggacgagctgcaggataagagcgagagcctgagcgataacgccaccgccttcagcaacagaagcaagcagctgcggagacagatgtggtggcggggctgcaagattaaggccatcatggctctggtggccgccatcctgctgctggtcatcatcatcctgatcgtgatgaagtaccggacaggcggcggaggatctggcggaggtggaagcggaggcggaggaagtggatctattggagccgccagcatggaattttgcttcgacgtgttcaaagaactgaaggtgcaccacgccaacgagaacatcttctactgccctatcgccatcatgagcgccctggctatggtgtatctgggcgccaaggacagcacccggacacagatcaacaaggtcgtcagattcgacaagctgcccggcttcggcgattctatcgaagcccagtgtggcaccagcgtgaacgtgcacagcagcctgagagacatcctgaatcagatcaccaagcctaacgacgtgtactccttcagcctggccagcagactgtacgccgaggaaagataccccatcctgcctgagtacctgcagtgcgtgaaagagctgtacagaggcggcctggaacctatcaacttccagacagccgccgaccaggccagagagctgatcaattcttgggtcgagagccagaccaacggcatcatcagaaacgtgctgcagcccagctccgtggattctcagacagccatggtgctggtcaacgccattgtgtttaaaggcctgtgggagaaaaccttcaaggacgaggacacccaggccatgcctttcagagtgacagagcaagagtccaagcctgtgcagatgatgtaccagatcggcctgtttagagtggcctccatggcctccgagaagatgaagatcctcgagctgcctttcgccagcggcaccatgtctatgctggtgctgctgcctgatgaggtgtccggactggaacagctcgagagcatcatcaacttcgagaagctgaccgagtggaccagcagcaacgtgatggaagaacggaagatcaaggtgtacctgcctcggatgaagatggaagagaagtacaacctgaccagcgtgctgatggctatgggcatcacagacgtgttctccagcagcgccaatctgagcggcatcagctctgccgagagcctgaagatttctcaggccgtgcatgctgcccacgccgagattaacgaagccggcagagaagttgtgggatctgccgaagcaggcgtggacgctgcttctgtgtctgaggaattccgggccgaccatccttttctgttctgcatcaagcacattgccaccaacgccgtgctgttctttggcagatgcgtgtccccttga

SEQ ID NO: 62 - DNA, 1503 bp, synthetic construct
  source 1..1503: mol_type = other DNA; note = VAMP8-OVA
atggaagaggctagtgaaggcggcggaaacgacagagtgcggaatctgcagtctgaggtggaaggcgtgaagaacatcatgacccagaacgtggaacggatcctggccagaggcgagaacctggaacacctgagaaacaagaccgaggacctggaagccaccagcgagcactttaagaccaccagccagaaggtggcccggaagttctggtggaagaatgtgaagatgatcgtgctgatctgcgtgatcgtgttcatcatcatcctgttcatcgtgctgttcgccaccggcgccttttctggcggcggaggatctggcggaggtggaagcggaggcggaggaagtggatctattggagccgccagcatggaattttgcttcgacgtgttcaaagaactgaaggtgcaccacgccaacgagaacatcttctactgccctatcgccatcatgagcgccctggctatggtgtatctgggcgccaaggacagcacccggacacagatcaacaaggtcgtcagattcgacaagctgcccggcttcggcgattctatcgaagcccagtgtggcaccagcgtgaacgtgcacagcagcctgagagacatcctgaatcagatcaccaagcctaacgacgtgtactccttcagcctggccagcagactgtacgccgaggaaagataccccatcctgcctgagtacctgcagtgcgtgaaagagctgtacagaggcggcctggaacctatcaacttccagacagccgccgaccaggccagagagctgatcaattcttgggtcgagagccagaccaacggcatcatcagaaacgtgctgcagcccagctccgtggattctcagacagccatggtgctggtcaacgccattgtgtttaaaggcctgtgggagaaaaccttcaaggacgaggacacccaggccatgcctttcagagtgacagagcaagagtccaagcctgtgcagatgatgtaccagatcggcctgtttagagtggcctccatggcctccgagaagatgaagatcctcgagctgcctttcgccagcggcaccatgtctatgctggtgctgctgcctgatgaggtgtccggactggaacagctcgagagcatcatcaacttcgagaagctgaccgagtggaccagcagcaacgtgatggaagaacggaagatcaaggtgtacctgcctcggatgaagatggaagagaagtacaacctgaccagcgtgctgatggctatgggcatcacagacgtgttctccagcagcgccaatctgagcggcatcagctctgccgagagcctgaagatttctcaggccgtgcatgctgcccacgccgagattaacgaagccggcagagaagttgtgggatctgccgaagcaggcgtggacgctgcttctgtgtctgaggaattccgggccgaccatccttttctgttctgcatcaagcacattgccaccaacgccgtgctgttctttggcagatgcgtgtccccttga

SEQ ID NO: 63 - DNA, 1899 bp, synthetic construct
  source 1..1899: mol_type = other DNA; note = VTI1B-OVA
atggctagctctgccgccagctctgagcacttcgagaagctgcacgagatcttcagaggcctgcacgaggacctgcagggcgttccagaaagactgctgggaacagccggcaccgaggaaaagaagaagctgatccgggacttcgacgagaagcagcaagaggccaatgagacactggccgagatggaagaggaactgagatacgcccctctgagcttcagaaaccccatgatgagcaagctgcggaactaccggaaggacctggccaagctgcatagagaagtgcggagcacccctctgacagctacacctggtggaagaggcgacatgaagtacggcatctacgccgtggaaaacgagcacatgaaccggctgcagagccagagagctatgctgctgcagggcaccgagagcctgaatagagccacacagagcatcgagcggagccacagaatcgccaccgagacagatcagatcggcagcgagatcatcgaggaactgggcgagcagagggaccagctggaaaggaccaagagcagactggtcaacaccagcgagaacctgagcaagagccggaagatcctgcggagcatgagcagaaaagtgaccaccaacaagctgctgctgagcatcatcatcctgctggaactggccatcctcggcggcctggtgtactacaagttcttcagaagccatggcggcggaggatctggcggaggtggaagcggaggcggaggaagtggatctattggagccgccagcatggaattttgcttcgacgtgttcaaagaactgaaggtgcaccacgccaacgagaacatcttctactgccctatcgccatcatgagcgccctggctatggtgtatctgggcgccaaggacagcacccggacacagatcaacaaggtcgtcagattcgacaagctgcccggcttcggcgattctatcgaagcccagtgtggcaccagcgtgaacgtgcacagcagcctgagagacatcctgaatcagatcaccaagcctaacgacgtgtactccttcagcctggccagcagactgtacgccgaggaaagataccccatcctgcctgagtacctgcagtgcgtgaaagagctgtacagaggcggcctggaacctatcaacttccagacagccgccgaccaggccagagagctgatcaattcttgggtcgagagccagaccaacggcatcatcagaaacgtgctgcagcccagctccgtggattctcagacagccatggtgctggtcaacgccattgtgtttaaaggcctgtgggagaaaaccttcaaggacgaggacacccaggccatgcctttcagagtgacagagcaagagtccaagcctgtgcagatgatgtaccagatcggcctgtttagagtggcctccatggcctccgagaagatgaagatcctcgagctgcctttcgccagcggcaccatgtctatgctggtgctgctgcctgatgaggtgtccggactggaacagctcgagagcatcatcaacttcgagaagctgaccgagtggaccagcagcaacgtgatggaagaacggaagatcaaggtgtacctgcctcggatgaagatggaagagaagtacaacctgaccagcgtgctgatggctatgggcatcacagacgtgttctccagcagcgccaatctgagcggcatcagctctgccgagagcctgaagatttctcaggccgtgcatgctgcccacgccgagattaacgaagccggcagagaagttgtgggatctgccgaagcaggcgtggacgctgcttctgtgtctgaggaattccgggccgaccatccttttctgttctgcatcaagcacattgccaccaacgccgtgctgttctttggcagatgcgtgtccccttga

SEQ ID NO: 64 - DNA, 1953 bp, synthetic construct
  source 1..1953: mol_type = other DNA; note = GOSR1-OVA
atggccgctggcacaagcagctactgggaagatctgcggaagcaggcccggcagctggaaaatgagctggacctgaagctggtgtccttcagcaagctgtgcaccagctacagccacagcagcaccagagatggcagacgggacagatacagcagcgacaccacacctctgctgaacggcagcagccaggaccggatgtttgagacaatggccatcgagatcgaacagctgctggccagactgaccggcgtgaacgataagatggccgagtacaccaactctgccggcgtgccaagtctgaacgccgctctgatgcacaccctgcagagacacagagacattctgcaggactacacccacgagttccacaagaccaaggccaacttcatggccattcgcgagcgcgagaatctgatgggctctgtgcggaaggacatcgagagctacaagagcggctctggcgtgaacaacagacggaccgagctgttcctgaaagagcacgaccacctgagaaacagcgaccggctgatcgaggaaaccatctctatcgccatggccaccaaagaaaacatgaccagccagcggggcatgctgaagtccatccacagcaagatgaacaccctggccaacagattccccgccgtgaacagcctgatccagcggatcaatctgagaaagcggcgggactctctgatcctcggcggagtgatcggcatctgtaccatcctgctgctgctctacgccttccatggcggcggaggatctggcggaggtggaagcggaggcggaggaagtggatctattggagccgccagcatggaattttgcttcgacgtgttcaaagaactgaaggtgcaccacgccaacgagaacatcttctactgccctatcgccatcatgagcgccctggctatggtgtatctgggcgccaaggacagcacccggacacagatcaacaaggtcgtcagattcgacaagctgcccggcttcggcgattctatcgaagcccagtgtggcaccagcgtgaacgtgcacagcagcctgagagacatcctgaatcagatcaccaagcctaacgacgtgtactccttcagcctggccagcagactgtacgccgaggaaagataccccatcctgcctgagtacctgcagtgcgtgaaagagctgtacagaggcggcctggaacctatcaacttccagacagccgccgaccaggccagagagctgatcaattcttgggtcgagagccagaccaacggcatcatcagaaacgtgctgcagcccagctccgtggattctcagacagccatggtgctggtcaacgccattgtgtttaaaggcctgtgggagaaaaccttcaaggacgaggacacccaggccatgcctttcagagtgacagagcaagagtccaagcctgtgcagatgatgtaccagatcggcctgtttagagtggcctccatggcctccgagaagatgaagatcctcgagctgcctttcgccagcggcaccatgtctatgctggtgctgctgcctgatgaggtgtccggactggaacagctcgagagcatcatcaacttcgagaagctgaccgagtggaccagcagcaacgtgatggaagaacggaagatcaaggtgtacctgcctcggatgaagatggaagagaagtacaacctgaccagcgtgctgatggctatgggcatcacagacgtgttctccagcagcgccaatctgagcggcatcagctctgccgagagcctgaagatttctcaggccgtgcatgctgcccacgccgagattaacgaagccggcagagaagttgtgggatctgccgaagcaggcgtggacgctgcttctgtgtctgaggaattccgggccgaccatccttttctgttctgcatcaagcacattgccaccaacgccgtgctgttctttggcagatgcgtgtccccttga

SEQ ID NO: 65 - DNA, 1557 bp, synthetic construct
  source 1..1557: mol_type = other DNA; note = BET1-OVA
atgcggagagccggacttggagaaggtgtccctcctggcaactacggcaattacggctacgccaacagcggctactctgcctgcgaggaagagaacgagagactgaccgagagcctgcggagcaaagtgaccgccatcaagagcctgagcatcgagatcggccacgaagtgaaaacccagaacaagctgctggccgagatggacagccagttcgacagcaccacaggctttctgggcaagaccatgggcaagctgaagatcctgagcagaggcagccagacaaagctgctgtgctacatgatgctgttcagcctgttcgtgttcttcatcatctactggatcatcaagctgagaggcggcggaggatctggcggaggtggaagcggaggcggaggaagtggatctattggagccgccagcatggaattttgcttcgacgtgttcaaagaactgaaggtgcaccacgccaacgagaacatcttctactgccctatcgccatcatgagcgccctggctatggtgtatctgggcgccaaggacagcacccggacacagatcaacaaggtcgtcagattcgacaagctgcccggcttcggcgattctatcgaagcccagtgtggcaccagcgtgaacgtgcacagcagcctgagagacatcctgaatcagatcaccaagcctaacgacgtgtactccttcagcctggccagcagactgtacgccgaggaaagataccccatcctgcctgagtacctgcagtgcgtgaaagagctgtacagaggcggcctggaacctatcaacttccagacagccgccgaccaggccagagagctgatcaattcttgggtcgagagccagaccaacggcatcatcagaaacgtgctgcagcccagctccgtggattctcagacagccatggtgctggtcaacgccattgtgtttaaaggcctgtgggagaaaaccttcaaggacgaggacacccaggccatgcctttcagagtgacagagcaagagtccaagcctgtgcagatgatgtaccagatcggcctgtttagagtggcctccatggcctccgagaagatgaagatcctcgagctgcctttcgccagcggcaccatgtctatgctggtgctgctgcctgatgaggtgtccggactggaacagctcgagagcatcatcaacttcgagaagctgaccgagtggaccagcagcaacgtgatggaagaacggaagatcaaggtgtacctgcctcggatgaagatggaagagaagtacaacctgaccagcgtgctgatggctatgggcatcacagacgtgttctccagcagcgccaatctgagcggcatcagctctgccgagagcctgaagatttctcaggccgtgcatgctgcccacgccgagattaacgaagccggcagagaagttgtgggatctgccgaagcaggcgtggacgctgcttctgtgtctgaggaattccgggccgaccatccttttctgttctgcatcaagcacattgccaccaacgccgtgctgttctttggcagatgcgtgtccccttga

SEQ ID NO: 66 - DNA, 2073 bp, synthetic construct
  source 1..2073: mol_type = other DNA; note = BET1L-OVA
atggccttttgcgccatcctgctggtgcctagcctgtgcagaatgcccagcctgcctacaagcccttgggcctttcctgtgcattgggccggcttcatgttcaagcccctggactggcagggcaacgacttcttcccacctcaagacgaagtgctggccccttgcctgggcatcaagacacctctgaagcacgagccctgtgctagcctgcctttcagcgtgctgtttcagagcagcgccagccagtctctgctgggcacaatgggatctctgagccctcacctgtgcggccacacaatgtgccctgtgaatcctgagctgccactgagcttccaggccgaccatagatctgcccagccagatgcctgcagtcccctgtgtcatccatctagcctgctgcctagcttccacaccgcttctctgcccttcagcattcacgcccaccactctccactgccttgcgaccttgatcctcctctgtacctggccgagacagtgtccctgctggaagaatggggacctcctagcagctgccccatgcagtgcaagctgacatctcaccctgccagactgacccatctgcctccatgtctgtggggctttgccgtggctctgaagccttcttgggctggccttgctccttctctgctgcctccacctagaatgagcctgtgtagacccctgtccttcctgcggcatcagtgtccttggctgccttggcaggctcaccaaggacttgttccttggagcccctctatggtggccgctgcctgtatcgtgtctcctagcggacactgtagatgccagcctttcatccctcacgtgttcctcggacacggcggcctgacatctgtgtctggcgaatgcggaggcggcggaggatctggcggaggtggaagcggaggcggaggaagtggatctattggagccgccagcatggaattttgcttcgacgtgttcaaagaactgaaggtgcaccacgccaacgagaacatcttctactgccctatcgccatcatgagcgccctggctatggtgtatctgggcgccaaggacagcacccggacacagatcaacaaggtcgtcagattcgacaagctgcccggcttcggcgattctatcgaagcccagtgtggcaccagcgtgaacgtgcacagcagcctgagagacatcctgaatcagatcaccaagcctaacgacgtgtactccttcagcctggccagcagactgtacgccgaggaaagataccccatcctgcctgagtacctgcagtgcgtgaaagagctgtacagaggcggcctggaacctatcaacttccagacagccgccgaccaggccagagagctgatcaattcttgggtcgagagccagaccaacggcatcatcagaaacgtgctgcagcccagctccgtggattctcagacagccatggtgctggtcaacgccattgtgtttaaaggcctgtgggagaaaaccttcaaggacgaggacacccaggccatgcctttcagagtgacagagcaagagtccaagcctgtgcagatgatgtaccagatcggcctgtttagagtggcctccatggcctccgagaagatgaagatcctcgagctgcctttcgccagcggcaccatgtctatgctggtgctgctgcctgatgaggtgtccggactggaacagctcgagagcatcatcaacttcgagaagctgaccgagtggaccagcagcaacgtgatggaagaacggaagatcaaggtgtacctgcctcggatgaagatggaagagaagtacaacctgaccagcgtgctgatggctatgggcatcacagacgtgttctccagcagcgccaatctgagcggcatcagctctgccgagagcctgaagatttctcaggccgtgcatgctgcccacgccgagattaacgaagccggcagagaagttgtgggatctgccgaagcaggcgtggacgctgcttctgtgtctgaggaattccgggccgaccatccttttctgttctgcatcaagcacattgccaccaacgccgtgctgttctttggcagatgcgtgtccccttga

SEQ ID NO: 67 - DNA, 1848 bp, synthetic construct
  source 1..1848: mol_type = other DNA; note = SEC22B-OVA
atggtcctgctgaccatgattgccagagtggccgatggactgcctctggccgctagcatgcaagaggatgagcagagcggcagagatctgcagcagtaccagtctcaggccaagcagctgttccggaagctgaacgagcagagccctaccagatgcacccttgaagccggcgctatgaccttccactacatcatcgagcagggcgtgtgctacctggtgctgtgcgaagccgcctttcctaagaagctggccttcgcctacctggaagatctgcacagcgagttcgatgagcagcacggcaagaaggtgcccaccgtcagcagaccctacagcttcatcgagttcgacaccttcatccaaaagaccaagaagctgtacatcgacagccgggccagaagaaacctgggcagcatcaataccgagctgcaggacgtgcagagaatcatggtggccaacatcgaggaagtgctgcagagaggcgaagccctgtctgccctggatagcaaggccaacaatctgagcagcctgagcaagaagtaccggcaggacgccaagtacctgaacatgagaagcacctacgccaagctggccgccgtggccgtgttcttcatcatgctgatcgtgtacgtgcggttctggtggcttggcggcggaggatctggcggaggtggaagcggaggcggaggaagtggatctattggagccgccagcatggaattttgcttcgacgtgttcaaagaactgaaggtgcaccacgccaacgagaacatcttctactgccctatcgccatcatgagcgccctggctatggtgtatctgggcgccaaggacagcacccggacacagatcaacaaggtcgtcagattcgacaagctgcccggcttcggcgattctatcgaagcccagtgtggcaccagcgtgaacgtgcacagcagcctgagagacatcctgaatcagatcaccaagcctaacgacgtgtactccttcagcctggccagcagactgtacgccgaggaaagataccccatcctgcctgagtacctgcagtgcgtgaaagagctgtacagaggcggcctggaacctatcaacttccagacagccgccgaccaggccagagagctgatcaattcttgggtcgagagccagaccaacggcatcatcagaaacgtgctgcagcccagctccgtggattctcagacagccatggtgctggtcaacgccattgtgtttaaaggcctgtgggagaaaaccttcaaggacgaggacacccaggccatgcctttcagagtgacagagcaagagtccaagcctgtgcagatgatgtaccagatcggcctgtttagagtggcctccatggcctccgagaagatgaagatcctcgagctgcctttcgccagcggcaccatgtctatgctggtgctgctgcctgatgaggtgtccggactggaacagctcgagagcatcatcaacttcgagaagctgaccgagtggaccagcagcaacgtgatggaagaacggaagatcaaggtgtacctgcctcggatgaagatggaagagaagtacaacctgaccagcgtgctgatggctatgggcatcacagacgtgttctccagcagcgccaatctgagcggcatcagctctgccgagagcctgaagatttctcaggccgtgcatgctgcccacgccgagattaacgaagccggcagagaagttgtgggatctgccgaagcaggcgtggacgctgcttctgtgtctgaggaattccgggccgaccatccttttctgttctgcatcaagcacattgccaccaacgccgtgctgttctttggcagatgcgtgtccccttga

SEQ ID NO: 68 - DNA, 1980 bp, synthetic construct
  source 1..1980: mol_type = other DNA; note = USE1-OVA
atggccgcctctagactggaactgaatctcgtgcggctgctgagcagatgcgaagctatggccgccgagaagagggaccctgatgaatggcggctcgagaaatatgtgggcgccctggaagatatgctgcaggccctgaaagtgcacgccagcaagcctgccagcgaagtgatcaacgagtacagctggaaggtggacttcctgaagggcatgctccaggccgagaagctgacaagcagctctgaaaaggccctggccaaccagtttctggcccctggtagagtgcctaccaccgccagagaaagagtgccagccaccaagacagtgcacctccagagcagagccagatacaccagcgagatgagaagcgagctgctgggcacagattctgccgagcctgaaatggacgtgcggaagagaacaggcgtggcaggctctcagcctgtgtccgaaaaacagctggccgctgagctggatctggtgctgcagagacaccagaacctgcaagagaagctggccgaggaaatgctgggcctcgccagatctctgaaaacaaacaccctggccgctcagagcgtgatcaagaaggacaatcagaccctgagccacagcctgaagatggccgaccagaatctggaaaagctgaaaaccgagagcgagcggctggaacagcacacccagaaaagcgtgaactggctgctgtgggccatgctgatcatcgtgtgcttcatcttcatcagcatgatcctgttcatccggatcatgcccaagctgaaaggcggcggaggatctggcggaggtggaagcggaggcggaggaagtggatctattggagccgccagcatggaattttgcttcgacgtgttcaaagaactgaaggtgcaccacgccaacgagaacatcttctactgccctatcgccatcatgagcgccctggctatggtgtatctgggcgccaaggacagcacccggacacagatcaacaaggtcgtcagattcgacaagctgcccggcttcggcgattctatcgaagcccagtgtggcaccagcgtgaacgtgcacagcagcctgagagacatcctgaatcagatcaccaagcctaacgacgtgtactccttcagcctggccagcagactgtacgccgaggaaagataccccatcctgcctgagtacctgcagtgcgtgaaagagctgtacagaggcggcctggaacctatcaacttccagacagccgccgaccaggccagagagctgatcaattcttgggtcgagagccagaccaacggcatcatcagaaacgtgctgcagcccagctccgtggattctcagacagccatggtgctggtcaacgccattgtgtttaaaggcctgtgggagaaaaccttcaaggacgaggacacccaggccatgcctttcagagtgacagagcaagagtccaagcctgtgcagatgatgtaccagatcggcctgtttagagtggcctccatggcctccgagaagatgaagatcctcgagctgcctttcgccagcggcaccatgtctatgctggtgctgctgcctgatgaggtgtccggactggaacagctcgagagcatcatcaacttcgagaagctgaccgagtggaccagcagcaacgtgatggaagaacggaagatcaaggtgtacctgcctcggatgaagatggaagagaagtacaacctgaccagcgtgctgatggctatgggcatcacagacgtgttctccagcagcgccaatctgagcggcatcagctctgccgagagcctgaagatttctcaggccgtgcatgctgcccacgccgagattaacgaagccggcagagaagttgtgggatctgccgaagcaggcgtggacgctgcttctgtgtctgaggaattccgggccgaccatccttttctgttctgcatcaagcacattgccaccaacgccgtgctgttctttggcagatgcgtgtccccttga

SEQ ID NO: 69 - DNA, 1881 bp, synthetic construct
  source 1..1881: mol_type = other DNA; note = VAMP7-pc-OVA
atggccatcctgttcgccgtggtggctagaggcacaaccattctggccaagcacgcttggtgcggcggcaactttctggaagtgaccgagcagatcctggccaagattcccagcgagaacaacaagctgacctacagccacggcaactacctgttccactacatctgccaggaccggatcgtgtacctgtgcatcaccgacgacgacttcgagcggagcagagccttcaacttcctgaacgagatcaagaagcggttccagaccacctacggcagcagagcacaaacagccctgccttacgccatgaacagcgagttcagctctgtgctggccgctcagctgaagcaccactccgagaacaaaggcctggacaaagtgatggaaacacaggcccaggtggacgagctgaagggcatcatggtccgaaacatcgacctggtggcccagagaggcgagagactggaactgctgatcgacaagaccgagaacctggtggacagcagcgtgaccttcaagaccaccagcagaaacctggccagagccatgtgcatgaagaacctgaagctgacgatcatcatcattatcgtgtccatcgtgttcatctacatcatcgtgtccccactgtgtggcggcttcacctggcctagctgtgtgaagaaatctggcggcggaggatctggcggaggtggaagcggaggcggtggatctagaagggccagaagaggatctatcggagccgccagcatggaattttgcttcgacgtgttcaaagaactgaaggtgcaccacgccaacgagaacatcttctactgccctatcgccatcatgagcgccctggctatggtgtatctgggcgccaaggacagcacccggacacagatcaacaaggtcgtcagattcgacaagctgcccggcttcggcgattctatcgaagcccagtgtggcaccagcgtgaacgtgcacagcagcctgagagacatcctgaatcagatcaccaagcctaacgacgtgtactccttcagcctggccagcagactgtacgccgaggaaagataccccatcctgcctgagtacctgcagtgcgtgaaagagctgtacagaggcggcctggaacctatcaacttccagacagccgccgaccaggccagagagctgatcaattcttgggtcgagagccagaccaacggcatcatcagaaacgtgctgcagcccagctccgtggattctcagacagccatggtgctggtcaacgccattgtgtttaaaggcctgtgggagaaaaccttcaaggacgaggacacccaggccatgcctttcagagtgacagagcaagagtccaagcctgtgcagatgatgtaccagatcggcctgtttagagtggcctccatggcctccgagaagatgaagatcctcgagctgcctttcgccagcggcaccatgtctatgctggtgctgctgcctgatgaggtgtccggactggaacagctcgagagcatcatcaacttcgagaagctgaccgagtggaccagcagcaacgtgatggaagaacggaagatcaaggtgtacctgcctcggatgaagatggaagagaagtacaacctgaccagcgtgctgatggctatgggcatcacagacgtgttctccagcagcgccaatctgagcggcatcagctctgccgagagcctgaagatttctcaggccgtgcatgctgcccacgccgagattaacgaagccggcagagaagttgtgggatctgccgaagcaggcgtggacgctgcttctgtgtctgaggaattccgggccgaccatccttttctgttctgcatcaagcacattgccaccaacgccgtgctgttctttggcagatgcgtgtccccttga

SEQ ID NO: 70 - DNA, 2409 bp, synthetic construct
  source 1..2409: mol_type = other DNA; note = LAMP[OVA]
atggctgcccctggctctgctagaaggcctctgctgttgctgcttctgctgctgctcctgggcctgatgcattgtgcctctgccgccatgttcatggtcaagaacggcaatggcaccgcctgcatcatggccaatttcagcgccgccttcagcgtgaactacgacaccaagagcggccccaagaacatgaccttcgacctgccttctgacgccaccgtggtgctgaatagaagcagctgcggcaaagagaacaccagcgatcccagcctcgtgatcgcctttggcagaggccatacactgaccctgaacttcacccggaacgccaccagatacagcgtgcagctgatgagcttcgtgtacaacctgagcgacacccatctgttccccaacgccagcagcaaagagatcaagaccgtcgagagcatcaccgacatccgggccgacatcgacaaaaagtacagatgcgtgtccggcacacaggtgcacatgaacaacgtgaccgtgacactgcacgacgccaccatccaggcctacctgagcaacagctctttcagcaggggcgagacaagatgcgagcaggacagaccctctcctaccactgctcctccagctccaccttctccaagtccatctcctgtgcctaagagccccagcgtggacaagtacaatgtgtctggcaccaacggcacctgtctgctggcttctatgggcctgcagctgaacctgacctacgagcggaaggacaacaccaccgtgaccagactgctgaacatcaaccccaacaagaccagcgccagcggatcttgtggcgcccatctggttacactggaactgcacagcgagggcaccacagtgctgctgttccagttcggcatgaacgccagctccagccggttcttcctgcaaggcatccagctgaacaccatcctgcctgacgccagagatcctgccttcaaggccgccaatggaagcctgagagcactgcaggccacagtgggcaacagctacaagtgcaacgccgaggaacacgtgcgcgtgaccaaggccttctccgtgaacatcttcaaagtgtgggtgcaagcctttaaggtggaaggcggccagtttggcagcgtggaagaatgcctgctggacgagaatagcatgggctctatcggagccgccagcatggaattttgcttcgacgtgttcaaagagctgaaggtccaccacgccaacgagaatatcttctactgccctatcgccatcatgagcgccctggccatggtgtatctgggcgccaaggatagcacccggacacagatcaacaaggtcgtcagattcgacaagctgcccggcttcggcgattctatcgaagcccagtgtggcacctccgtgaatgtgcacagcagcctgagggacatcctgaaccagatcaccaagcctaacgacgtgtacagcttcagcctggcctccagactgtacgccgaagagagataccccattctgcccgagtacctgcagtgtgtgaaagaactgtacagaggcggcctggaacctatcaacttccagacagccgccgaccaggccagagagctgatcaattcttgggtcgagagccagaccaatggcatcatccggaacgtgctgcagcccagctctgtggattctcagactgccatggtgctggtcaacgccatcgtgtttaaaggcctgtgggagaaaaccttcaaggacgaggacacccaggccatgcctttcagagtgaccgagcaagagtccaagcctgtgcagatgatgtaccagatcggcctgtttagagtggcctccatggcctccgagaagatgaagatcctcgagctgcctttcgccagcggcaccatgtctatgttggtgctgctgcccgatgaggtgtccggactggaacaactggaatccatcatcaacttcgagaagctgaccgagtggaccagctccaacgtgatggaagaacggaagatcaaggtgtacctgcctcggatgaagatggaagagaagtacaatctgaccagcgtgctgatggccatgggaatcaccgatgtgttctccagcagcgccaacctgtctggcatcagctctgccgagagcctgaagatttctcaggccgtgcatgccgctcacgccgagatcaatgaagccggcagagaagttgtgggatctgccgaagcaggcgtggacgctgcatctgtgtctgaggaattcagagccgaccatccttttctgttctgcatcaagcacattgccaccaacgccgtgctgttcttcggaagatgtgtgtcccctctgatcccaatcgccgttggaggtgctctggctggactggtgctgatcgtgctgattgcctacctcgtgggcagaaagagaagccacgccggctaccagaccatctga

SEQ ID NO: 71 - DNA, 753 bp, Homo sapiens
  source 1..753: mol_type = genomic DNA
atggcggcagggaccagcagttactgggaagatctcaggaaacaggctcgacagctggaaaatgaacttgacctgaaactagtttccttcagcaaactatgtacaagttacagtcatagcagtacccgagatggaagacgcgacaggtatagttctgatacaacaccccttttaaatggatcaagccaagacagaatgtttgagacaatggcgattgagattgaacaacttttggcaaggcttacaggggtaaatgataaaatggcagaatataccaacagtgcaggtgtcccctccttgaatgcagccctgatgcatacattacagcggcatagagacatattgcaggattatacacatgaattccataaaaccaaagcaaactttatggcaatacgggaaagggagaatcttatgggatcagtacgaaaagatattgagtcatataaaagtgggtctggagtaaacaacagaagaactgagctatttttgaaagaacatgaccaccttcgaaactcagatcgtctgatagaagagacaataagcattgctatggcaacaaaagaaaatatgacttcacagagaggaatgttgaagtcaattcacagcaaaatgaacactttggccaatcgttttcctgctgtaaacagcctgatccagaggatcaacctgaggaagcggcgggactcgctcatcctagggggtgttattgggatctgtaccatcctgttgctgctgtatgcgttccattga

SEQ ID NO: 72 - DNA, 711 bp, Homo sapiens
  source 1..711: mol_type = genomic DNA
atggcaccggacccctggttctccacatacgattctacttgtcaaattgcccaagaaattgctgagaaaattcaacaacgaaatcaatatgaaagaaaaggtgaaaaggcaccaaagcttaccgtgacaatcagagctttgttgcagaacctgaaggaaaagatcgcccttttgaaggacttattgctaagagctgtgtcaacacatcagataacacagcttgaaggggaccgaagacagaacctcttggatgatcttgtaactcgagagagactacttctggcatcctttaagaatgagggtgccgaaccagatctaatcaggtccagcctgatgagtgaagaggctaagcgaggagcacccaacccttggctctttgaggagccagaggagaccagaggcttgggttttgatgaaatccggcaacagcagcagaaaattatccaagaacaggacgcaggccttgatgccctttcctctatcataagtcgccaaaaacaaatggggcaggaaattgggaatgaattggatgaacaaaatgagataattgacgaccttgccaacctagtggagaacacagatgaaaaacttcgcaatgaaaccaggcgggtaaacatggtggacagaaagtcagcctcttgtgggatgatcatggtgattttactgctgcttgtggctatcgtggttgttgcagtctggccgaccaactga

SEQ ID NO: 73 - DNA, 831 bp, Homo sapiens
  source 1..831: mol_type = genomic DNA
atgtcatacggtcccttagacatgtaccggaacccggggccctcggggccccagctccgggacttcagcagcatcatccagacgtgcagcggcaacatccagcggatcagccaagccactgctcagataaagaatttgatgagccagctaggaactaagcaggactcaagcaagctacaggaaaatctgcaacagttacaacactccacaaatcagctcgccaaggaaacaaatgaattgctgaaagaattagggtccttgccccttcccttatctacttcagaacagcgccagcagagacttcagaaggaacgcctcatgaatgacttctctgcagccttaaacaatttccaggctgtgcagagaagggtatctgaaaaggaaaaggagagtattgccagagcaagagctggatctcgtctttctgcagaagagaggcaaagagaggagcagctggtctcatttgacagccatgaggagtggaaccagatgcagagccaggaggatgaggtggccatcactgagcaggatttggaacttattaaagaaagagaaacggcaattcggcagctggaggctgacattttggatgtcaatcagatatttaaagatttggccatgatgatccatgaccagggtgatctgattgatagcatagaagccaatgtggaaagctcagaggtgcacgtcgaaagagccactgaacagttacagcgagctgcttactatcagaaaaaatctcgcaagaagatgtgtatcctggtgcttgtcctgtcagtgattattctaatcttgggacttattatctggctagtttataaaacgaagtga

SEQ ID NO: 74 - DNA, 303 bp, Homo sapiens
  source 1..303: mol_type = genomic DNA
atggaggaagccagtgaaggtggaggaaatgatcgtgtgcggaacctgcaaagtgaggtggagggagttaagaatattatgacccagaatgtggagcggatcctggcccggggggaaaacttggaacatctccgcaacaagacagaggatctggaagccacatctgagcacttcaagacgacatcgcagaaggtggctcgaaaattctggtggaagaacgtgaagatgattgtccttatctgcgtgattgtttttatcatcatcctcttcattgtgctctttgccactggtgccttctcttaa

SEQ ID NO: 75 - DNA, 648 bp, Homo sapiens
  source 1..648: mol_type = genomic DNA
atggtgttgctaacaatgatcgcccgagtggcggacgggctcccgctggccgcctcgatgcaggaggacgaacagtctggccgggaccttcaacaatatcagagtcaggctaagcaactctttcgaaagttgaatgaacagtcccctaccagatgtaccttggaagcaggagccatgacttttcactacattattgagcagggggtgtgttatttggttttatgtgaagctgccttccctaagaagttggcttttgcctacctagaagatttgcactcagaatttgatgaacagcatggaaagaaggtgcccactgtgtcccgaccctattcctttattgaatttgatactttcattcagaaaaccaagaagctctacattgacagtcgtgctcgaagaaatctaggctccatcaacactgaattgcaagatgtgcagaggatcatggtggccaatattgaagaagtgttacaacgaggagaagcactctcagcattggattcaaaggctaacaatttgtccagtctgtccaagaaataccgccaggatgcgaagtacttgaacatgcgttccacttatgccaaacttgcagcagtagctgtatttttcatcatgttaatagtgtatgtccgattctggtggctgtga

SEQ ID NO: 76 - protein, 250 aa, Homo sapiens
MAAGTSSYWEDLRKQARQLENELDLKLVSFSKLCTSYSHSSTRDGRRDRYSSDTTPLLNGSSQDRMFETMAIEIEQLLARLTGVNDKMAEYTNSAGVPSLNAALMHTLQRHRDILQDYTHEFHKTKANFMAIRERENLMGSVRKDIESYKSGSGVNNRRTELFLKEHDHLRNSDRLIEETISIAMATKENMTSQRGMLKSIHSKMNTLANRFPAVNSLIQRINLRKRRDSLILGGVIGICTILLLLYAFH

SEQ ID NO: 77 - protein, 236 aa, Homo sapiens
MAPDPWFSTYDSTCQIAQEIAEKIQQRNQYERKGEKAPKLTVTIRALLQNLKEKIALLKDLLLRAVSTHQITQLEGDRRQNLLDDLVTRERLLLASFKNEGAEPDLIRSSLMSEEAKRGAPNPWLFEEPEETRGLGFDEIRQQQQKIIQEQDAGLDALSSIISRQKQMGQEIGNELDEQNEIIDDLANLVENTDEKLRNETRRVNMVDRKSASCGMIMVILLLLVAIVVVAVWPTN

SEQ ID NO: 78 - protein, 276 aa, Homo sapiens
MSYGPLDMYRNPGPSGPQLRDFSSIIQTCSGNIQRISQATAQIKNLMSQLGTKQDSSKLQENLQQLQHSTNQLAKETNELLKELGSLPLPLSTSEQRQQRLQKERLMNDFSAALNNFQAVQRRVSEKEKESIARARAGSRLSAEERQREEQLVSFDSHEEWNQMQSQEDEVAITEQDLELIKERETAIRQLEADILDVNQIFKDLAMMIHDQGDLIDSIEANVESSEVHVERATEQLQRAAYYQKKSRKKMCILVLVLSVIILILGLIIWLVYKTK

SEQ ID NO: 79 - protein, 100 aa, Homo sapiens
MEEASEGGGNDRVRNLQSEVEGVKNIMTQNVERILARGENLEHLRNKTEDLEATSEHFKTTSQKVARKFWWKNVKMIVLICVIVFIIILFIVLFATGAFS

SEQ ID NO: 80 - protein, 215 aa, Homo sapiens
MVLLTMIARVADGLPLAASMQEDEQSGRDLQQYQSQAKQLFRKLNEQSPTRCTLEAGAMTFHYIIEQGVCYLVLCEAAFPKKLAFAYLEDLHSEFDEQHGKKVPTVSRPYSFIEFDTFIQKTKKLYIDSRARRNLGSINTELQDVQRIMVANIEEVLQRGEALSALDSKANNLSSLSKKYRQDAKYLNMRSTYAKLAAVAVFFIMLIVYVRFWWL

SEQ ID NO: 81 - DNA, 1161 bp, synthetic construct
  source 1..1161: mol_type = other DNA
atgggctctatcggagccgccagcatggaattttgcttcgacgtgttcaaagagctgaaggtccaccacgccaacgagaacatcttctactgccctatcgccatcatgagcgccctggccatggtgtatctgggcgccaaggatagcacccggacacagatcaacaaggtcgtcagattcgacaagctgcccggcttcggcgattctatcgaagcccagtgtggcaccagcgtgaacgtgcacagcagcctgagagacatcctgaaccagatcaccaagcctaacgacgtgtacagcttcagcctggccagcagactgtacgccgaggaaagataccccatcctgcctgagtacctgcagtgcgtgaaagagctgtacagaggcggcctggaacctatcaacttccagacagccgccgaccaggccagagagctgatcaattcttgggtcgagagccagaccaacggcatcatcagaaacgtgctgcagcccagctccgtggattctcagacagccatggtgctggtcaacgccatcgtgtttaaaggcctgtgggagaaaaccttcaaggacgaggacacccaggccatgcctttcagagtgaccgagcaagagtccaagcctgtgcagatgatgtaccagatcggcctgtttagagtggcctccatggcctccgagaagatgaagatcctggaactgcctttcgccagcggcaccatgtctatgctggtgctgctgcctgatgaggtgtccggactggaacagctggaatccatcatcaacttcgagaagctgaccgagtggaccagcagcaacgtgatggaagaacggaagatcaaggtgtacctgcctcggatgaagatggaagagaagtacaacctgaccagcgtgctgatggccatgggaatcaccgatgtgttcagcagcagcgccaacctgagcggcattagctctgccgagagcctgaagattagccaggccgtgcatgctgcccacgccgagatcaatgaagccggcagagaagttgtgggatctgccgaagcaggcgtggacgctgcttctgtgtctgaggaattccgggccgaccatccttttctgttctgcatcaagcacattgccaccaacgccgtgctgttctttggcagatgcgtgtccccttga

SEQ ID NO: 82 - DNA, 1290 bp, Homo sapiens
  source 1..1290: mol_type = genomic DNA
atgggctccgacgtgcgggacctgaacgcgctgctgcccgccgtcccctccctgggtggcggcggcggctgtgccctgcctgtgagcggcgcggcgcagtgggcgccggtgctggactttgcgcccccgggcgcttcggcttacgggtcgttgggcggccccgcgccgccaccggctccgccgccacccccgccgccgccgcctcactccttcatcaaacaggagccgagctggggcggcgcggagccgcacgaggagcagtgcctgagcgccttcactgtccacttttccggccagttcactggcacagccggagcctgtcgctacgggcccttcggtcctcctccgcccagccaggcgtcatccggccaggccaggatgtttcctaacgcgccctacctgcccagctgcctcgagagccagcccgctattcgcaatcagggttacagcacggtcaccttcgacgggacgcccagctacggtcacacgccctcgcaccatgcggcgcagttccccaaccactcattcaagcatgaggatcccatgggccagcagggctcgctgggtgagcagcagtactcggtgccgcccccggtctatggctgccacacccccaccgacagctgcaccggcagccaggctttgctgctgaggacgccctacagcagtgacaatttataccaaatgacatcccagcttgaatgcatgacctggaatcagatgaacttaggagccaccttaaagggccacagcacagggtacgagagcgataaccacacaacgcccatcctctgcggagcccaatacagaatacacacgcacggtgtcttcagaggcattcaggatgtgcgacgtgtgcctggagtagccccgactcttgtacggtcggcatctgagaccagtgagaaacgccccttcatgtgtgcttacccaggctgcaataagagatattttaagctgtcccacttacagatgcacagcaggaagcacactggtgagaaaccataccagtgtgacttcaaggactgtgaacgaaggttttctcgttcagaccagctcaaaagacaccaaaggagacatacaggtgtgaaaccattccagtgtaaaacttgtcagcgaaagttctcccggtccgaccacctgaagacccacaccaggactcatacaggtgaaaagcccttcagctgtcggtggccaagttgtcagaaaaagtttgcccggtcagatgaattagtccgccatcacaacatgcatcagagaaacatgaccaaactccagctggcgctttga

SEQ ID NO: 83 - DNA, 1290 bp, synthetic construct
  source 1..1290: mol_type = other DNA
atgggcagcgacgtgcgggatctgaatgctctgcttcctgccgtgccatctcttggcggaggcggaggatgtgctttgcctgtttctggtgctgcccagtgggctcccgtgctggattttgctcctcctggcgcctctgcctatggctctcttggaggacctgctcctccaccagctccacctccaccgccgcctccaccacctcacagctttatcaagcaagagccctcctggggcggagccgaacctcatgaagaacagtgcctgagcgccttcaccgtgcacttcagcggacagtttacaggcacagccggcgcttgtagatacggcccttttggaccacctcctccaagccaggcttctagcggacaagcccggatgttccccaacgctccttacctgcctagctgcctggaaagccagcctgccatcagaaaccagggctacagcaccgtgaccttcgatggcacacctagctacggccacacaccatctcatcacgccgctcagttccccaatcacagcttcaagcacgaggaccctatgggccagcagggatctctgggagagcagcagtatagcgtgccacctcctgtgtacggctgtcacacccctaccgatagctgtacaggatctcaggccctgctgctgagaaccccttacagcagcgacaacctgtaccagatgaccagccagctggaatgcatgacctggaaccagatgaacctgggcgccacactgaagggccacagcacaggctacgagtccgacaaccacaccacacctattctgtgcggagcccagtaccggatccacacacatggcgtgttcagaggcatccaggacgtgcgaagagtgcctggcgttgcccctacactcgtcagatctgccagcgagacaagcgagaagcgccccttcatgtgtgcctatcctggctgcaacaagcggtacttcaagctgagccacctccagatgcacagcagaaagcacaccggcgagaagccctaccagtgcgacttcaaggactgcgagcggcggttcagcagaagcgaccagctgaaaagacaccagcggaggcacacaggcgtgaaacctttccagtgcaagacctgccagcggaagttctccagatccgatcacctgaaaacccacacacggacccacacaggggagaagccattcagctgtagatggcccagctgccagaagaagttcgctcggagcgacgaactcgtgcggcaccacaatatgcaccagagaaacatgaccaaactgcagctggccctgtga

SEQ ID NO: 84 - protein, 429 aa, Homo sapiens
MGSDVRDLNALLPAVPSLGGGGGCALPVSGAAQWAPVLDFAPPGASAYGSLGGPAPPPAPPPPPPPPPHSFIKQEPSWGGAEPHEEQCLSAFTVHFSGQFTGTAGACRYGPFGPPPPSQASSGQARMFPNAPYLPSCLESQPAIRNQGYSTVTFDGTPSYGHTPSHHAAQFPNHSFKHEDPMGQQGSLGEQQYSVPPPVYGCHTPTDSCTGSQALLLRTPYSSDNLYQMTSQLECMTWNQMNLGATLKGHSTGYESDNHTTPILCGAQYRIHTHGVFRGIQDVRRVPGVAPTLVRSASETSEKRPFMCAYPGCNKRYFKLSHLQMHSRKHTGEKPYQCDFKDCERRFSRSDQLKRHQRRHTGVKPFQCKTCQRKFSRSDHLKTHTRTHTGEKPFSCRWPSCQKKFARSDELVRHHNMHQRNMTKLQLAL

SEQ ID NO: 85 - DNA, 444 bp, synthetic construct
  source 1..444: mol_type = other DNA
atggaggtgggttggtaccgttctcccttctcaagagtggttcacctctaccgaaatggcaagatggaggtgggttggtaccgttctcccttctcaagagtggttcacctctaccgaaatggcaagatggaggtgggttggtaccgttctcccttctcaagagtggttcacctctaccgaaatggcaagatggaggtgggttggtaccgttctcccttctcaagagtggttcacctctaccgaaatggcaagatggaggtgggttggtaccgttctcccttctcaagagtggttcacctctaccgaaatggcaagatggaggtgggttggtaccgttctcccttctcaagagtggttcacctctaccgaaatggcaagatggaggtgggttggtaccgttctcccttctcaagagtggttcacctctaccgaaatggcaagtga

SEQ ID NO: 86 - DNA, 444 bp, synthetic construct
  source 1..444: mol_type = other DNA
atggaagtcggctggtatagaagccccttcagcagagtggtgcacctgtaccggaacggcaagatggaagttggatggtacaggtccccattcagccgggtcgtgcatctgtatagaaatggaaagatggaagttggctggtatcggagcccattttccagggtcgtccacctctacagaaacggcaaaatggaagtcggctggtacagatctccattctctagagtggtccatctctatcgcaacggaaagatggaagtcggatggtatcgctcccctttctctcgcgtggtgcatctttatcggaatggcaaaatggaagttggctggtataggtccccgttctccagagtcgttcacttgtataggaacggaaaaatggaagttggatggtatagatcacccttctctagggttgtgcacctctataggaatgggaagtga

SEQ ID NO: 87 - protein, 147 aa, synthetic construct
MEVGWYRSPFSRVVHLYRNGKMEVGWYRSPFSRVVHLYRNGKMEVGWYRSPFSRVVHLYRNGKMEVGWYRSPFSRVVHLYRNGKMEVGWYRSPFSRVVHLYRNGKMEVGWYRSPFSRVVHLYRNGKMEVGWYRSPFSRVVHLYRNGK

SEQ ID NO: 88 - DNA, 2010 bp, synthetic construct
  source 1..2010: mol_type = other DNA; note = VAMP7-pc-WT1
atggccatcctgttcgccgtggtggctagaggcacaaccattctggccaagcacgcttggtgcggcggcaactttctggaagtgaccgagcagatcctggccaagattcccagcgagaacaacaagctgacctacagccacggcaactacctgttccactacatctgccaggaccggatcgtgtacctgtgcatcaccgacgacgacttcgagcggagcagagccttcaacttcctgaacgagatcaagaagcggttccagaccacctacggcagcagagcacaaacagccctgccttacgccatgaacagcgagttcagctctgtgctggccgctcagctgaagcaccactccgagaacaaaggcctggacaaagtgatggaaacacaggcccaggtggacgagctgaagggcatcatggtccgaaacatcgacctggtggcccagagaggcgagagactggaactgctgatcgacaagaccgagaacctggtggacagcagcgtgaccttcaagaccaccagcagaaacctggccagagccatgtgcatgaagaacctgaagctgacgatcatcatcattatcgtgtccatcgtgttcatctacatcatcgtgtccccactgtgtggcggcttcacctggcctagctgtgtgaagaaatctggcggcggaggatctggcggaggtggaagcggaggcggtggatctagaagggctagaagaggctccgacgtgcgggacctgaatgctctgcttcctgccgtgccatctcttggcggtggtggtggatgtgcactgcctgtttctggtgctgctcagtgggctcccgtgctggattttgctcctcctggcgcctctgcctatggctctcttggaggacctgctcctccaccagctccaccgccacctccgcctccaccacctcacagctttatcaagcaagagccctcctggggcggagccgaacctcacgaagaacagtgtctgagcgccttcaccgtgcacttcagcggccagtttactggaacagccggcgcttgtagatacggcccttttggacctccacctcctagccaggcatctagcggacaggccaggatgttccccaacgctccttacctgccaagctgcctggaaagccagcctgccatcagaaaccagggctacagcaccgtgacattcgacggcacacctagctacggccacacaccttctcatcacgccgctcagttccccaatcacagcttcaagcacgaggaccccatgggccagcaaggatctttgggcgagcagcagtacagcgtgccacctcctgtgtacggctgtcacacccctaccgatagctgtacaggatctcaggccctgctgctgagaaccccttacagcagcgacaacctgtaccagatgaccagccagctggaatgcatgacctggaaccagatgaacctgggcgccacactgaagggccacagcacaggctacgagtccgacaaccacaccacacctattctgtgcggagcccagtaccggatccacacacatggcgtgttcagaggcatccaggacgtgcgaagagtgcctggcgttgcccctacactcgtcagatctgccagcgagacaagcgagaagcgccccttcatgtgtgcctatcctggctgcaacaagcggtacttcaagctgagccacctccagatgcacagcagaaagcacaccggcgagaagccctaccagtgcgacttcaaggactgcgagaggcggttcagcagaagcgaccagctgaagagacaccagcggagacatacaggcgtgaagcctttccagtgcaagacctgccagcggaagttctccagatccgaccacctgaaaacccacacaagaacccacaccggggaaaagccattcagctgcagatggcccagctgccagaagaagttcgctcggagcgacgaactcgtgcggcaccacaatatgcaccagagaaacatgaccaaactgcagctggccctgtga

SEQ ID NO: 89 - protein, 669 aa, synthetic construct
  source 1..669: note = VAMP7-pc-WT1
MAILFAVVARGTTILAKHAWCGGNFLEVTEQILAKIPSENNKLTYSHGNYLFHYICQDRIVYLCITDDDFERSRAFNFLNEIKKRFQTTYGSRAQTALPYAMNSEFSSVLAAQLKHHSENKGLDKVMETQAQVDELKGIMVRNIDLVAQRGERLELLIDKTENLVDSSVTFKTTSRNLARAMCMKNLKLTIIIIIVSIVFIYIIVSPLCGGFTWPSCVKKSGGGGSGGGGSGGGGSRRARRGSDVRDLNALLPAVPSLGGGGGCALPVSGAAQWAPVLDFAPPGASAYGSLGGPAPPPAPPPPPPPPPHSFIKQEPSWGGAEPHEEQCLSAFTVHFSGQFTGTAGACRYGPFGPPPPSQASSGQARMFPNAPYLPSCLESQPAIRNQGYSTVTFDGTPSYGHTPSHHAAQFPNHSFKHEDPMGQQGSLGEQQYSVPPPVYGCHTPTDSCTGSQALLLRTPYSSDNLYQMTSQLECMTWNQMNLGATLKGHSTGYESDNHTTPILCGAQYRIHTHGVFRGIQDVRRVPGVAPTLVRSASETSEKRPFMCAYPGCNKRYFKLSHLQMHSRKHTGEKPYQCDFKDCERRFSRSDQLKRHQRRHTGVKPFQCKTCQRKFSRSDHLKTHTRTHTGEKPFSCRWPSCQKKFARSDELVRHHNMHQRNMTKLQLAL

SEQ ID NO: 90 - DNA, 1167 bp, synthetic construct
  source 1..1167: mol_type = other DNA; note = VAMP7-pc-MOG 35-55
atggccatcctgttcgccgtggtggctagaggcacaaccattctggccaagcacgcttggtgcggcggcaactttctggaagtgaccgagcagatcctggccaagattcccagcgagaacaacaagctgacctacagccacggcaactacctgttccactacatctgccaggaccggatcgtgtacctgtgcatcaccgacgacgacttcgagcggagcagagccttcaacttcctgaacgagatcaagaagcggttccagaccacctacggcagcagagcacaaacagccctgccttacgccatgaacagcgagttcagctctgtgctggccgctcagctgaagcaccactccgagaacaaaggcctggacaaagtgatggaaacacaggcccaggtggacgagctgaagggcatcatggtccgaaacatcgacctggtggcccagagaggcgagagactggaactgctgatcgacaagaccgagaacctggtggacagcagcgtgaccttcaagaccaccagcagaaacctggccagagccatgtgcatgaagaacctgaagctgacgatcatcatcattatcgtgtccatcgtgttcatctacatcatcgtgtccccactgtgtggcggcttcacctggcctagctgtgtgaagaaatctggcggcggaggatctggcggaggtggaagcggaggcggtggatctagacgggctagaagaatggaagtcggctggtatcggagccccttcagcagagtggtgcacctgtaccggaacggcaagatggaagttggatggtacaggtccccattcagccgggtcgtgcatctgtatagaaatggaaagatggaagttggctggtatcgctctccattctccagagtggtccatctctaccgcaatggaaaaatggaagtcggatggtatagaagcccattctccagggttgtgcacctctacagaaacggaaaaatggaagtcggctggtacagatctcccttctctcgcgtggtgcatctttatcgcaacggaaagatggaagtcggatggtatcggtcaccttttagccgcgttgtccacctgtatcgtaatggcaaaatggaagttggatggtatcgctcacccttcagccgagtggttcatctctacagaaatggcaagtga

SEQ ID NO: 91 - protein, 388 aa, synthetic construct
  source 1..388: note = VAMP7-pc-MOG 35-55
MAILFAVVARGTTILAKHAWCGGNFLEVTEQILAKIPSENNKLTYSHGNYLFHYICQDRIVYLCITDDDFERSRAFNFLNEIKKRFQTTYGSRAQTALPYAMNSEFSSVLAAQLKHHSENKGLDKVMETQAQVDELKGIMVRNIDLVAQRGERLELLIDKTENLVDSSVTFKTTSRNLARAMCMKNLKLTIIIIIVSIVFIYIIVSPLCGGFTWPSCVKKSGGGGSGGGGSGGGGSRRARRMEVGWYRSPFSRVVHLYRNGKMEVGWYRSPFSRVVHLYRNGKMEVGWYRSPFSRVVHLYRNGKMEVGWYRSPFSRVVHLYRNGKMEVGWYRSPFSRVVHLYRNGKMEVGWYRSPFSRVVHLYRNGKMEVGWYRSPFSRVVHLYRNGK

SEQ ID NO: 92 - protein, 4 aa, synthetic construct
  REGION >4: note = The entire sequences of amino acids 1-4 can be repeated one to five times.
GGGS

SEQ ID NO: 93 - protein, 5 aa, synthetic construct
  REGION >5: note = The entire sequences of amino acids 1-5 can be repeated one to five times.
GGGGS

SEQ ID NO: 94 - protein, 5 aa, synthetic construct
  REGION >5: note = The entire sequences of amino acids 1-5 can be repeated one to five times.
EAAAK